European Patent Specification EP 3 826 671 B1, published August 14, 2024. Title: NOUVELLE SOUCHE VIRALE ATTENUEE ET SON UTILISATION EN TANT QUE VACCIN. Applicant: UNIVERSITE CLAUDE BERNARD LYON 1 CENTRE NATIONAL DE LA RECHERCHE SCIENTIFIQUE (CNRS) ECOLE NORMALE SUPERIEURE DE LYON INSTITUT NATIONAL DE LA SANTE ET DE LA RECHERCHE MEDICALE (INSERM) UNIVERSITE LAVAL. The sequence listing filed with the application follows.

SEQUENCE LISTING (8 sequences)

SEQ ID NO: 1 - DNA, 13394 bp, metapneumovirus
gcgaaaaaaacgcgtataaattagattacaaaaaaatatgggacaagtgaaaatgtctcttcaagggattcacctgagtgatctatcatacaagcatgctatattaaaagagtctcagtacacaataaaaagagatgtgggtacaacaactgcagtgacaccctcatcattgcaacaagaaataacgctgttgtgtggagaaattctgtatgctaaacatgctgattacaaatatgctgcagaaataggaatacaatatattagcacagctttaggatcagagagagtgcagcagattctgaggaactcaggcagtgaagtccaagtggtcttaaccagaacgtactctctggggaaagttaaaaacaataaaggagaagatttacagatgttagacatacacggggtagagaagagctgggtagaagagatagacaaagaagcaaggaaaacaatggcaaccttgcttaaggaatcatcaggtaatatcccacaaaatcagaggccctcagcaccagacacacccataatcttattatgtgtaggtgcattaatatttactaagctagcatcaaccatagaagtgggactagagaccacagtcagaagggctaaccgtgtactaagtgatgcactcaagagataccctagaatggacatcccaaaaattgccagatccttctatgacttatttgaacaaaaagtgtatcacagaagtttgttcattgagtatggcaaagcattaggctcatcatctacaggcagcaaagcagaaagtctatttgttaatatattcatgcaagcttatggagccggtcaaacaatgctaaggtggggggtcattgccaggtcatccaacaatataatgttaggacatgtatctgtccaagctgagttaaaacaggtcacagaagtctatgacttggtgcgagaaatgggccctgaatctggacttctacatttaaggcaaagcccaaaagctggactgttatcactagccaactgtcccaactttgcaagtgttgttctcggaaatgcctcaggcttaggcataatcggtatgtatcgtgggagagtaccaaacacagaattattttcagcagcagaaagttatgccaaaagtttgaaagagagcaataaaatcaatttctcttcattaggacttacagatgaagagaaagaggctgcagaacatttcttaaatgtgagtgacgacagtcaaaatgattatgagtaattaaaaaagtgggacaagtcaaaatgtctttccctgaaggaaaagatattcttttcatgggtaatgaagcagcaaaattagcagaagctttccagaaatcattaaggaaaccaagtcataaaagatctcaatctattataggagaaaaagtgaacactgtatcagaaacattggaattacctactatcagtagacctgcaaaaccaaccatactgtcagaaccaaagttagcatggactgataaaggtggggcaatcaaaactgaaataaagcaagcaatcaaagtcatggatcctattgaggaagaagagtctactgagaagaaggtgctgccctccagtgatgggaaaacccctgcagaaaagaaactgaaaccatcaactaacaccaaaaagaaagtttcgtttacaccaaatgaaccaggaaaatatacaaagttggaaaaagatgctctagatttgctctcagataatgaagaagaagatgcagaatcttcaatcttaacctttgaagaaagagatacttcatcgttaagcattgaggccagattggaatcaatagaggagaaattaagcatgatattagggctattaagaacactcaacattgctacagcaggacccacagcagcaagagatgggatcagagatgcaatgattggcgtaagagaggaattaatagcagacataataaaggaagccaaagggaaagcagcagaaatgatggaagaggaaatgagtcaacgatcaaaaataggaaacggtagtgtaaaactaacagagaaagcaaaagagcttaacaaaattgttgaagatgaaagcacaagtggagaatctgaagaagaagaagaaccaaaagacatacaagacaatagtcaagaagatgacatttaccagttaattatgtagtttaataaaaataaacaatgggacaagtaaaaatggagtcctacctagtagacacttatcaaggcattccttacacagcagctgttcaagttgatctaatagaaaaggacctgttacctgcaagcctaacaatatggttccctttgtttcaggccaacacaccaccagcagtgctgctcgatcagttgaaaaccctaacaataaccactctgtatgctgcatcacaaaatggtccaatactcaaagtgaatgcatcagcccaaggtgcagcaatgtctgtacttcccaaaaaatttgaagtcaatgcgactgtagcactcgatgaatatagcaaattggaatttgacaaactcacagtctgtgaagtaaaaacagtttacttaacaaccatgaaaccatacgggatggtatcaaaatttgtgagctcagccaaatcagttggcaaaaaaacacatgatctaatcgcactgtgtgattttatggatctagaaaagaacacacctgttacaataccagcattcatcaaatcagtttcaatcaaagagagtgagtcagctactgttgaagctgctataagcagtgaagcagaccaagctctaacacaggccaaaattgcaccttatgcgggattgattatgatcatgactatgaacaatcccaaaggcatattcaaaaagcttggagctgggactcaagttatagtagaactaggagcatatgtccaggctgaaagcataagtaaaatatgcaagacttggagccatcaagggacaagatatgtgttgaagtccagataacagccaagcaccttggccaagagctactaactctatctcatagattataaagtcaccattctagttatataaaaatcaagttagaacaagaattaaatcaatcaagaatgggacaaataaaaatgtcttggaaagtggtgatcattttttcattgttaataacacctcaacacggtcttaaagagagctatttagaagagtcatgtagcactataactgaaggatatctcagtgttctgaggacaggttggtataccaacgtttttacactggaggtaggtgatgtagagaaccttacatgtgctgatggacctagcttaataaaaacagaattagacctgaccaaaagtgcactaagagaactcagaacagtttctgctgatcaactggcaagagaggagcaaattgagaatcccagacaatctagatttgttctaggagcaatagcactcggtgttgcaacagcagctgcagttacagcaggtgttgcaattgccaaaaccatccggcttgaaagtgaagtaacagcaattaagaatgccctcaaaaagaccaatgaagcagtatctacattggggaatggagttcgagtgttggcaactgcagtgagggagctggaagattttgtgagcaagaatctaacacgtgcaatcaacaaaaacaagtgcgacattgctgacctgaaaatggccgttagcttcagtcaattcaacagaaggtttctaaatgttgtgcggcaattttcagacaatgctggaataacaccagcaatatccttggacttaatgacagatgctgaactagccagagctgtttccaacatgccaacatctgcaggacaaataaaactgatgttggagaaccgtgcaatggtaagaagaaaggggttcggaatcctgataggagtttacggaagctccgtaatttacatggtgcaactgccaatctttggagttatagacacgccttgctggatagtaaaagcggccccttcttgctcagaaaaaaagggaaactatgcttgccttttaagagaagatcaaggatggtattgtcagaatgcagggtcaactgtttactacccaaatgaaaaagactgcgaaacaagaggagaccatgtcttttgcgacacagcagcaggaatcaatgttgctgagcagtcaaaggagtgcaacatcaacatatccactactaattacccatgcaaagttagcacaggaagacaccctatcagtatggttgcactgtctcctcttggggctttggttgcttgctacaagggagtgagctgttccattggcagcaacagagtagggatcatcaagcaactgaacaaaggctgctcttatataaccaaccaagacgcagacacagtgacaatagacaacactgtataccagctaagcaaagttgagggcgaacagcatgttataaaaggaaggccagtgtcaagcagctttgatccagtcaaatttcctgaagatcaattcaatgttgcacttgaccaagttttcgaaagcattgagaacagtcaggccttggtggatcaatcaaacagaatcctaagcagtgcagagaaaggaaacactggcttcatcattgtaataattctaattgctgtccttggctctaccatgatcctagtgagtgtttttatcataataaagaaaacaaagaaacccacaggagcacctccagagctgagtggtgtcacaaacaatggcttcataccacataattagttaattaaaaataaagtaaattaaattaaaataaaataaaattaaaattaaaataaaataaaaataaaaatttgggacaaatcataatgtctcgcaaggctccatgcaaatatgaagtgcggggcaaatgcaatagaggaagtgagtgcaagtttaaccacaattactggagttggccagatagatacttactaataagatcaaattatttattaaatcaacttttaaggaacactgatagagctgatggcttatcaataatatcaggagcaggcagagaagataggacacaagattttgtcctaggttccaccaatgtggttcaaggttatattgatgataaccaaagcataacaaaagctgcagcctgttacagtctacataatataatcaaacaactacaagaagttgaagttaggcaggctagagataacaaaccatctgacagcaaacatgtggcacttcacaacttagtcctatcttatatggagatgagcaaaattcctgcatctttaatcaacaatctcaaaagactgccgagagagaaactgaaaaaattagcaaagcttataattgacttatcagcaggtgctgaaaatgactcttcatatgccttgcaagacagtgaaagcactaatcaagtgcagtgagcatggtcctgttttcattactatagaggttgattacatgatatggactcataaggacttaaaagaagctttatctaatgggatagtgaagtctcatactaacatttacaattgttatttagaaaacatagaaattatatatgtcaaggcttacttaagttagtaaaaacacatcagagtgggataaatgacaatgataacattagatgtcattaaaagtgatgggtcttcaaaaacatgtactcacctcaaaaaattaattaaagaccactctggtaaagtgcttattgtacttaagttaatattagctttactaacatttctcacagtgacaatcaccatcaattatataaaagtagaaaacaatctgcaaatatgtcagtcaaaaactgaatcagacaaaaaggactcatcatcaaataccacatcagtcacaaccaagactactctaaatcatgatataacacagtattttaaaagtttgattcaaaggtatacaaactctgcaataaacagagacacatgctggaaaataagcagaaatcaatgcacaaacataacaacatacaaatttttatgttttaaatctgaagaaacaaaaaccaacaattgtgataaactgacagatttatgcagaaacaaaccaaaaccagctgttgaagtgtatcacatagtagaatgccattgtatatacacagttaaatggaagtgctatcattacccaatagatgaaacccaatcctaaataacactagattaggatccatccaagtctgttagttcaacaatttagttatttaaaaatattttgaaaacaagtaagtttctatgatacttcataataataagtaataattaattgcttaatcatcatcacaacattattcgaaaccataactattcaatttaagaagtaaaaacaataatatgggacaagtagttatggaggtgaaagtggagaacattcgaacaatagatatgctcaaagcaagagtgaaaaatcgtgtggcacgcagcaaatgctttaaaaatgcctctttgatcctaataggaataactacattgagtatagccctcaatatctatctaatcataaactatacaatgcaagaaaacacatccgaatcagaacatcacaccagctcatcacccatggaatccagcagggaaactccaacagtccctatggacaactcagacaccaatccaggctcacagtatccaactcaacagtccacagaaggctccacactctactttgcagcctcagcaagctcaccagagacagaaccaacatcaacaccagacacaacaagccgcccgcccttcgtcgacacacacacaacactaccaagtgcaagcagaacaaggacaagtccggcagtccacacaaaaaacaatccaaggacaagccccagaacacattccccaccatgggcaatgacaaggacggtccgtggaaccaccactctccgcacaagcagcacaagaaaaagaccgtccacagcatcagtccaacctgacagcagcgcaacaacccacaaacacgaagaagcaagcccagtgagcccgcaaacatctgcgagcacagcaagaccacaaaggaagggcatggaggccagcacatcaacaacatacaaccaaactagttaacaaaaaatacaaaataactctaagataaaccatatagacaccaacaattgagaagccaaaaggcaattcacaatctctccaaaaaggcaacaacaccatattagctccgcttaaatctccctggaaaaaacactcgcccatataccaactataccacaaccatcccaagaaaaaaagctgggtaaaacaacacccaagagacaaataacaatggatcctcttaatgaatccactgttaatgtctatcttcccgactcatatcttaaaggagtgatttcttttagtgagactaatgcaattggttcatgtctcttaaaaagaccttacctaaaaaatgacaacactgcaaaagttgccatagagaatcctgttatcgagcatgttagactcaaaaatgcaatcaattctaagatgaaaatatcagattacaggatagtagagccagtaaacatgcaacatgaaattatgaagaatgtacacagttgtgagctcacattattaaaacagtttttaacaaggagtaaaaatattagcactcttaaattaaatatgatatgtgattggctgcagttaaagtctacatcagatgatacctcaatcttaagttttatagatgtagaatttatacctagctgggtaagcaattggtttagtaattggtacaatctcaacaagttgattctggaattcaggaaagaagaagtaataagaactggttcaatcttgtgtaggtcattgggtaaattagtttttgttgtatcatcatacggatgtatagtcaagagcaacaaaagcaaaagagtgagcttcttcacatacaatcaactgttaacatggaaagatgtgatgttaagtagattcaatgcaaatttctgtatatgggtaagcaacagtctgaatgaaaatcaagaagggttagggttgagaagtaatctgcaaggcatattaactaataagctatatgaaactgtagattatatgcttagtttgtgttgcaatgaaggtttctcacttgtgaaagagtttgagggttttattatgagtgaaatccttaggattactgaacatgctcaattcagtactagatttagaaatactttattaaatggattaactgatcaattgacaaaattaaaaaataaaaacagactcagagttcatggtaccgtgttagaaaataatgattatccaatgtatgaagttgtacttaaattattaggagatactttgagatgtattaaattattaatcaataaaaacttagagaatgctgctgaattatactatatatttagaatattcggtcacccaatggtagatgaaagagatgcaatggatgctgtcaaattaaacaatgaaatcacaaaaatcctcaggttggagagcttgacagaactaagaggggcattcatattaaggattatcaaaggatttgtagacaacaacaaaagatggccgaaaattaaaaacttaaaagtgcttagtaaaagatggactatgtacttcaaagcaaaaagttaccctagtcaacttgaattaagtgaacaagattttttagagcttgctgcaatacagtttgaacaagagttttctgttcctgaaaaaaccaaccttgagatggtattaaatgataaagctatatcacctcctaaaagattaatttggtctgtgtacccaaaaaattacttacctgagacaataaaaaatcgatatctagaagagactttcaatgcaagtgatagtctcaaaacaagaagagtactagagtactatttgaaagataataaattcgaccaaaaagaacttaaaagttatgtggttaaacaagaatatttaaatgataaggatcatattgtctcgctaactggaaaagaaagagaattaagtgtaggtagaatgtttgctatgcaaccaggaaaacagcgacaaatacaaatattggctgaaaaattgttagctgataatattgtaccctttttcccagaaactttaacaaagtatggtgatctagatcttcagagaataatggaaatcaaatcagaactttcttctattaaaaccagaagaaatgatagttataataattacattgcaagagcatccatagtaacagatttaagtaagttcaaccaagcctttaggtatgaaactacagcgatctgtgcggatgtagcagatgaactacatggaacacaaagcctattctgttggttacatcttatcgttcctatgactacaatgatatgtgcctatagacatgcaccaccagaaacaaaaggtgaatatgatatagataagatagaagagcaaagtggtttatatagatatcatatgggtggtattgaaggatggtgtcaaaaactctggacaatggaagctatatctttattagatgttgtatctgtaaagacacgatgtcaaatgacatctttattaaacggtgacaaccaatcaatagatgtaagtaaaccagttaagttatctgagggtttagatgaagtgaaagcagattatagcttggctgtaaaaatgctaaaagaaataagagatgcatacagaaatataggccataaacttaaagaaggggaaacatatatatcaagagatcttcagtttataagtaaggtgattcaatctgaaggagtaatgcatcctacccctataaaaaagatcttaagagtgggaccatggataaacacaatattagatgacattaaaaccagtgcagagtcaatagggagtctatgtcaggaattagaatttaggggggaaagcataatagttagtctgatattaaggaatttttggctgtataatttatacatgcatgaatcaaagcaacaccccctagcagggaagcagttattcaaacaactaaataaaacattaacatcagtgcagagattttttgaaattaaaaaggaaaatgaagtagtagatctatggatgaacataccaatgcagtttggaggaggagatccagtagtcttctatagatctttctatagaaggacccctgattttttaactgaagcaatcagtcatgtagatattctgttaaaaatatcagccaacataagaaatgaagcgaaaataagtttcttcaaagccttactgtcaatagaaaaaaatgaacgtgctacactgacaacactaatgagagaccctcaagctgtgggctcagagcgacaagcaaaagtaacaagtgatatcaatagaacagcagttaccagcatcttaagtctttctccaaatcaacttttcagcgatagtgctatacactacagtagaaatgaagaagaggtcggaatcattgctgacaacataacacctgtttatcctcatggactgagagttttgtatgaatcattaccttttcataaagctgaaaaagttgtaaatatgatatcaggaacaaaatccataaccaacttattacagagaacatctgctattaatggtgaagatattgacagagctgtatccatgatgctggagaacctaggattattatctagaatattgtcagtagttgttgatagtatagaaattccaaccaaatctaatggtaggctgatatgttgtcagatatctagaaccctaagggagacatcatggaataatatggaaatagttggagtaacatcccctagcatcactacatgcatggatgtcatatatgcaactagctctcatttgaaagggataatcattgaaaagttcagcactgacagaactacaagaggtcaaagaggtccaaagagcccttgggtaggatcgagcacgcaagagaaaaaattagttcctgtttataacagacaaattctttcaaaacaacaaagagaacagctagaagcaattggaaaaatgagatgggtatataaagggacaccaggtttaagacgattactcaataagatttgtcttggaagtttaggcattagttacaaatgtgtaaaacctttattacctaggtttatgagtgtaaatttcctacacaggttatctgtcagtagtagacctatggaattcccagcatcagttccagcttatagaacaacaaattaccattttgacactagtcctattaatcaagcactaagtgaaagatttgggaatgaagatattaatttggtcttccaaaatgcaatcagctgtggaattagcataatgagtgtagtagaacaattaactggtaggagtccaaaacagttagttttaataccccaattagaagaaatagacattatgccaccaccagtgtttcaagggaaattcaattataagctagtagataagataacttctgaccaacatatcttcagtccagacaaaatagatatgttaacactggggaaaatgctcatgccaactataaaaggtcagaaaacagatcagttcttgaacaagagagagaattatttccatgggaacaatcttattgagtctttgtcagcagcgttagcatgtcattggtgtgggatattaacagagcaatgtatagaaaataatattttcaagaaagactggggtgacgggttcatatcggatcatgcttttatggacttcaaaatattcctatgtgtctttaaaactaaacttttatgtagttggggatcccaagggaaaaacattaaagatgaagatatagtagatgaatcgatagataaactgttaaggattgataatactttttggagaatgttcagcaaggttatgtttgaatcaaaggttaagaaaaggataatgttatatgatgtaaaatttctatcattagtaggttatatagggtttaagaattggtttatagaacagttgagatcagctgagttgcatgaggtaccttggattgtcaatgccgaaggtgatctggttgagatcaagtcaattaaaatctatttgcaactgatagagcagagtttatttttaagaataactgttttgaactatacagatatggcacatgctctcacaagattaatcagaaagaagttgatgtgtgataatgcactattaacttcaattccatccccaatggttaacttaactcaagttattgatcctacagaacaattagcttatttccctaagataacatttgaaaggctaaaaaattatgacactagttcaaattatgctaaaggaaagctaacaaggaattacatgatactgttgccatggcaacatgttaatagatataactttgtctttagttctactggatgtaaagttagtctaaaaacatgcattggaaaacttatgaaagatctaaaccctaaagttctgtactttattggagaaggggcaggaaattggatggccagaacagcatgtgaatatcctgacatcaaatttgtatacagaagtttaaaagatgaccttgatcatcattatcctttggaataccagagagtgataggagaattaagcaggataatagatagtggtgaagggctttcaatggaaacaacagatgcaactcaaaaaactcattgggatttgatacacagagtaagcaaagatgctttattaataactttatgtgatgcagaatttaaggacagagatgatttttttaagatggtaattctatggaggaaacatgtattatcatgcagaatttgcactacctatgggacagacctctatttattcgcaaagtatcatgctaaagactgcaatataaaattacctttttttgtgagatcagttgccacctttattatgcaaggtagtaaactgtcaggctcggaatgctacatactcttaacactaggccaccacaacaatttaccttgtcatggagaaatacaaaattctaagatgaaaatagcagcgtgtaatgatttttatgctgcaaaaaaacttgacaataaatcaattgaagccaactgtaaatcacttttatcagggctaagaataccgataaataagaaggaattaaatagacagagaaggttattaacactacaaagcaaccattcttctgtagcaacagttggaggtagcaaggtcatagagtctaaatggttaacaaacaaggcaaacacaataattgattggttagaacatattttaaattctccaaaaggtgaattaaattatgatttttttgaagcattagaaaatacttaccctaatatgattaaactaatagataatctagggaatgcagagattaaaaaactgatcaaagtaactggatatatgcttgtaagtaaaaaatgaaaaatgataaaaatgataaaataggtgacaacttcatactattccaaagtaatcatttgattatgcaattatgtaatagttaattaaaaactaaaaatcaaaagttaaaaactaataactgtcattaagtttattaaaaataagaaattataattggatgtatacggtttttttgccgt

SEQ ID NO: 2 - DNA, 12645 bp, metapneumovirus
gcgaaaaaaacgcgtataaattagattacaaaaaaatatgggacaagtgaaaatgtctcttcaagggattcacctgagtgatctatcatacaagcatgctatattaaaagagtctcagtacacaataaaaagagatgtgggtacaacaactgcagtgacaccctcatcattgcaacaagaaataacgctgttgtgtggagaaattctgtatgctaaacatgctgattacaaatatgctgcagaaataggaatacaatatattagcacagctttaggatcagagagagtgcagcagattctgaggaactcaggcagtgaagtccaagtggtcttaaccagaacgtactctctggggaaagttaaaaacaataaaggagaagatttacagatgttagacatacacggggtagagaagagctgggtagaagagatagacaaagaagcaaggaaaacaatggcaaccttgcttaaggaatcatcaggtaatatcccacaaaatcagaggccctcagcaccagacacacccataatcttattatgtgtaggtgcattaatatttactaagctagcatcaaccatagaagtgggactagagaccacagtcagaagggctaaccgtgtactaagtgatgcactcaagagataccctagaatggacatcccaaaaattgccagatccttctatgacttatttgaacaaaaagtgtatcacagaagtttgttcattgagtatggcaaagcattaggctcatcatctacaggcagcaaagcagaaagtctatttgttaatatattcatgcaagcttatggagccggtcaaacaatgctaaggtggggggtcattgccaggtcatccaacaatataatgttaggacatgtatctgtccaagctgagttaaaacaggtcacagaagtctatgacttggtgcgagaaatgggccctgaatctggacttctacatttaaggcaaagcccaaaagctggactgttatcactagccaactgtcccaactttgcaagtgttgttctcggaaatgcctcaggcttaggcataatcggtatgtatcgtgggagagtaccaaacacagaattattttcagcagcagaaagttatgccaaaagtttgaaagagagcaataaaatcaatttctcttcattaggacttacagatgaagagaaagaggctgcagaacatttcttaaatgtgagtgacgacagtcaaaatgattatgagtaattaaaaaagtgggacaagtcaaaatgtctttccctgaaggaaaagatattcttttcatgggtaatgaagcagcaaaattagcagaagctttccagaaatcattaaggaaaccaagtcataaaagatctcaatctattataggagaaaaagtgaacactgtatcagaaacattggaattacctactatcagtagacctgcaaaaccaaccatactgtcagaaccaaagttagcatggactgataaaggtggggcaatcaaaactgaaataaagcaagcaatcaaagtcatggatcctattgaggaagaagagtctactgagaagaaggtgctgccctccagtgatgggaaaacccctgcagaaaagaaactgaaaccatcaactaacaccaaaaagaaagtttcgtttacaccaaatgaaccaggaaaatatacaaagttggaaaaagatgctctagatttgctctcagataatgaagaagaagatgcagaatcttcaatcttaacctttgaagaaagagatacttcatcgttaagcattgaggccagattggaatcaatagaggagaaattaagcatgatattagggctattaagaacactcaacattgctacagcaggacccacagcagcaagagatgggatcagagatgcaatgattggcgtaagagaggaattaatagcagacataataaaggaagccaaagggaaagcagcagaaatgatggaagaggaaatgagtcaacgatcaaaaataggaaacggtagtgtaaaactaacagagaaagcaaaagagcttaacaaaattgttgaagatgaaagcacaagtggagaatctgaagaagaagaagaaccaaaagacatacaagacaatagtcaagaagatgacatttaccagttaattatgtagtttaataaaaataaacaatgggacaagtaaaaatggagtcctacctagtagacacttatcaaggcattccttacacagcagctgttcaagttgatctaatagaaaaggacctgttacctgcaagcctaacaatatggttccctttgtttcaggccaacacaccaccagcagtgctgctcgatcagttgaaaaccctaacaataaccactctgtatgctgcatcacaaaatggtccaatactcaaagtgaatgcatcagcccaaggtgcagcaatgtctgtacttcccaaaaaatttgaagtcaatgcgactgtagcactcgatgaatatagcaaattggaatttgacaaactcacagtctgtgaagtaaaaacagtttacttaacaaccatgaaaccatacgggatggtatcaaaatttgtgagctcagccaaatcagttggcaaaaaaacacatgatctaatcgcactgtgtgattttatggatctagaaaagaacacacctgttacaataccagcattcatcaaatcagtttcaatcaaagagagtgagtcagctactgttgaagctgctataagcagtgaagcagaccaagctctaacacaggccaaaattgcaccttatgcgggattgattatgatcatgactatgaacaatcccaaaggcatattcaaaaagcttggagctgggactcaagttatagtagaactaggagcatatgtccaggctgaaagcataagtaaaatatgcaagacttggagccatcaagggacaagatatgtgttgaagtccagataacagccaagcaccttggccaagagctactaactctatctcatagattataaagtcaccattctagttatataaaaatcaagttagaacaagaattaaatcaatcaagaatgggacaaataaaaatgtcttggaaagtggtgatcattttttcattgttaataacacctcaacacggtcttaaagagagctatttagaagagtcatgtagcactataactgaaggatatctcagtgttctgaggacaggttggtataccaacgtttttacactggaggtaggtgatgtagagaaccttacatgtgctgatggacctagcttaataaaaacagaattagacctgaccaaaagtgcactaagagaactcagaacagtttctgctgatcaactggcaagagaggagcaaattgagaatcccagacaatctagatttgttctaggagcaatagcactcggtgttgcaacagcagctgcagttacagcaggtgttgcaattgccaaaaccatccggcttgaaagtgaagtaacagcaattaagaatgccctcaaaaagaccaatgaagcagtatctacattggggaatggagttcgagtgttggcaactgcagtgagggagctggaagattttgtgagcaagaatctaacacgtgcaatcaacaaaaacaagtgcgacattgctgacctgaaaatggccgttagcttcagtcaattcaacagaaggtttctaaatgttgtgcggcaattttcagacaatgctggaataacaccagcaatatccttggacttaatgacagatgctgaactagccagagctgtttccaacatgccaacatctgcaggacaaataaaactgatgttggagaaccgtgcaatggtaagaagaaaggggttcggaatcctgataggagtttacggaagctccgtaatttacatggtgcaactgccaatctttggagttatagacacgccttgctggatagtaaaagcggccccttcttgctcagaaaaaaagggaaactatgcttgccttttaagagaagatcaaggatggtattgtcagaatgcagggtcaactgtttactacccaaatgaaaaagactgcgaaacaagaggagaccatgtcttttgcgacacagcagcaggaatcaatgttgctgagcagtcaaaggagtgcaacatcaacatatccactactaattacccatgcaaagttagcacaggaagacaccctatcagtatggttgcactgtctcctcttggggctttggttgcttgctacaagggagtgagctgttccattggcagcaacagagtagggatcatcaagcaactgaacaaaggctgctcttatataaccaaccaagacgcagacacagtgacaatagacaacactgtataccagctaagcaaagttgagggcgaacagcatgttataaaaggaaggccagtgtcaagcagctttgatccagtcaaatttcctgaagatcaattcaatgttgcacttgaccaagttttcgaaagcattgagaacagtcaggccttggtggatcaatcaaacagaatcctaagcagtgcagagaaaggaaacactggcttcatcattgtaataattctaattgctgtccttggctctaccatgatcctagtgagtgtttttatcataataaagaaaacaaagaaacccacaggagcacctccagagctgagtggtgtcacaaacaatggcttcataccacataattagttaattaaaaataaagtaaattaaattaaaataaaataaaattaaaattaaaataaaataaaaataaaaatttgggacaaatcataatgtctcgcaaggctccatgcaaatatgaagtgcggggcaaatgcaatagaggaagtgagtgcaagtttaaccacaattactggagttggccagatagatacttactaataagatcaaattatttattaaatcaacttttaaggaacactgatagagctgatggcttatcaataatatcaggagcaggcagagaagataggacacaagattttgtcctaggttccaccaatgtggttcaaggttatattgatgataaccaaagcataacaaaagctgcagcctgttacagtctacataatataatcaaacaactacaagaagttgaagttaggcaggctagagataacaaaccatctgacagcaaacatgtggcacttcacaacttagtcctatcttatatggagatgagcaaaattcctgcatctttaatcaacaatctcaaaagactgccgagagagaaactgaaaaaattagcaaagcttataattgacttatcagcaggtgctgaaaatgactcttcatatgccttgcaagacagtgaaagcactaatcaagtgcagtgagcatggtcctgttttcattactatagaggttgattacatgatatggactcataaggacttaaaagaagctttatctaatgggatagtgaagtctcatactaacatttacaattgttatttagaaaacatagaaattatatatgtcaaggcttacttaagttagtaaaaacacatcagagtgggacaagtagttatggaggtgaaagtggagaacattcgaacaatagatatgctcaaagcaagagtgaaaaatcgtgtggcacgcagcaaatgctttaaaaatgcctctttgatcctaataggaataactacattgagtatagccctcaatatctatctaatcataaactatacaatgcaagaaaacacatccgaatcagaacatcacaccagctcatcacccatggaatccagcagggaaactccaacagtccctatggacaactcagacaccaatccaggctcacagtatccaactcaacagtccacagaaggctccacactctactttgcagcctcagcaagctcaccagagacagaaccaacatcaacaccagacacaacaagccgcccgcccttcgtcgacacacacacaacactaccaagtgcaagcagaacaaggacaagtccggcagtccacacaaaaaacaatccaaggacaagccccagaacacattccccaccatgggcaatgacaaggacggtccgtggaaccaccactctccgcacaagcagcacaagaaaaagaccgtccacagcatcagtccaacctgacagcagcgcaacaacccacaaacacgaagaagcaagcccagtgagcccgcaaacatctgcgagcacagcaagaccacaaaggaagggcatggaggccagcacatcaacaacatacaaccaaactagttaacaaaaaatacaaaataactctaagataaaccatatagacaccaacaattgagaagccaaaaggcaattcacaatctctccaaaaaggcaacaacaccatattagctccgcttaaatctccctggaaaaaacactcgcccatataccaactataccacaaccatcccaagaaaaaaagctgggtaaaacaacacccaagagacaaataacaatggatcctcttaatgaatccactgttaatgtctatcttcccgactcatatcttaaaggagtgatttcttttagtgagactaatgcaattggttcatgtctcttaaaaagaccttacctaaaaaatgacaacactgcaaaagttgccatagagaatcctgttatcgagcatgttagactcaaaaatgcaatcaattctaagatgaaaatatcagattacaggatagtagagccagtaaacatgcaacatgaaattatgaagaatgtacacagttgtgagctcacattattaaaacagtttttaacaaggagtaaaaatattagcactcttaaattaaatatgatatgtgattggctgcagttaaagtctacatcagatgatacctcaatcttaagttttatagatgtagaatttatacctagctgggtaagcaattggtttagtaattggtacaatctcaacaagttgattctggaattcaggaaagaagaagtaataagaactggttcaatcttgtgtaggtcattgggtaaattagtttttgttgtatcatcatacggatgtatagtcaagagcaacaaaagcaaaagagtgagcttcttcacatacaatcaactgttaacatggaaagatgtgatgttaagtagattcaatgcaaatttctgtatatgggtaagcaacagtctgaatgaaaatcaagaagggttagggttgagaagtaatctgcaaggcatattaactaataagctatatgaaactgtagattatatgcttagtttgtgttgcaatgaaggtttctcacttgtgaaagagtttgagggttttattatgagtgaaatccttaggattactgaacatgctcaattcagtactagatttagaaatactttattaaatggattaactgatcaattgacaaaattaaaaaataaaaacagactcagagttcatggtaccgtgttagaaaataatgattatccaatgtatgaagttgtacttaaattattaggagatactttgagatgtattaaattattaatcaataaaaacttagagaatgctgctgaattatactatatatttagaatattcggtcacccaatggtagatgaaagagatgcaatggatgctgtcaaattaaacaatgaaatcacaaaaatcctcaggttggagagcttgacagaactaagaggggcattcatattaaggattatcaaaggatttgtagacaacaacaaaagatggccgaaaattaaaaacttaaaagtgcttagtaaaagatggactatgtacttcaaagcaaaaagttaccctagtcaacttgaattaagtgaacaagattttttagagcttgctgcaatacagtttgaacaagagttttctgttcctgaaaaaaccaaccttgagatggtattaaatgataaagctatatcacctcctaaaagattaatttggtctgtgtacccaaaaaattacttacctgagacaataaaaaatcgatatctagaagagactttcaatgcaagtgatagtctcaaaacaagaagagtactagagtactatttgaaagataataaattcgaccaaaaagaacttaaaagttatgtggttaaacaagaatatttaaatgataaggatcatattgtctcgctaactggaaaagaaagagaattaagtgtaggtagaatgtttgctatgcaaccaggaaaacagcgacaaatacaaatattggctgaaaaattgttagctgataatattgtaccctttttcccagaaactttaacaaagtatggtgatctagatcttcagagaataatggaaatcaaatcagaactttcttctattaaaaccagaagaaatgatagttataataattacattgcaagagcatccatagtaacagatttaagtaagttcaaccaagcctttaggtatgaaactacagcgatctgtgcggatgtagcagatgaactacatggaacacaaagcctattctgttggttacatcttatcgttcctatgactacaatgatatgtgcctatagacatgcaccaccagaaacaaaaggtgaatatgatatagataagatagaagagcaaagtggtttatatagatatcatatgggtggtattgaaggatggtgtcaaaaactctggacaatggaagctatatctttattagatgttgtatctgtaaagacacgatgtcaaatgacatctttattaaacggtgacaaccaatcaatagatgtaagtaaaccagttaagttatctgagggtttagatgaagtgaaagcagattatagcttggctgtaaaaatgctaaaagaaataagagatgcatacagaaatataggccataaacttaaagaaggggaaacatatatatcaagagatcttcagtttataagtaaggtgattcaatctgaaggagtaatgcatcctacccctataaaaaagatcttaagagtgggaccatggataaacacaatattagatgacattaaaaccagtgcagagtcaatagggagtctatgtcaggaattagaatttaggggggaaagcataatagttagtctgatattaaggaatttttggctgtataatttatacatgcatgaatcaaagcaacaccccctagcagggaagcagttattcaaacaactaaataaaacattaacatcagtgcagagattttttgaaattaaaaaggaaaatgaagtagtagatctatggatgaacataccaatgcagtttggaggaggagatccagtagtcttctatagatctttctatagaaggacccctgattttttaactgaagcaatcagtcatgtagatattctgttaaaaatatcagccaacataagaaatgaagcgaaaataagtttcttcaaagccttactgtcaatagaaaaaaatgaacgtgctacactgacaacactaatgagagaccctcaagctgtgggctcagagcgacaagcaaaagtaacaagtgatatcaatagaacagcagttaccagcatcttaagtctttctccaaatcaacttttcagcgatagtgctatacactacagtagaaatgaagaagaggtcggaatcattgctgacaacataacacctgtttatcctcatggactgagagttttgtatgaatcattaccttttcataaagctgaaaaagttgtaaatatgatatcaggaacaaaatccataaccaacttattacagagaacatctgctattaatggtgaagatattgacagagctgtatccatgatgctggagaacctaggattattatctagaatattgtcagtagttgttgatagtatagaaattccaaccaaatctaatggtaggctgatatgttgtcagatatctagaaccctaagggagacatcatggaataatatggaaatagttggagtaacatcccctagcatcactacatgcatggatgtcatatatgcaactagctctcatttgaaagggataatcattgaaaagttcagcactgacagaactacaagaggtcaaagaggtccaaagagcccttgggtaggatcgagcacgcaagagaaaaaattagttcctgtttataacagacaaattctttcaaaacaacaaagagaacagctagaagcaattggaaaaatgagatgggtatataaagggacaccaggtttaagacgattactcaataagatttgtcttggaagtttaggcattagttacaaatgtgtaaaacctttattacctaggtttatgagtgtaaatttcctacacaggttatctgtcagtagtagacctatggaattcccagcatcagttccagcttatagaacaacaaattaccattttgacactagtcctattaatcaagcactaagtgaaagatttgggaatgaagatattaatttggtcttccaaaatgcaatcagctgtggaattagcataatgagtgtagtagaacaattaactggtaggagtccaaaacagttagttttaataccccaattagaagaaatagacattatgccaccaccagtgtttcaagggaaattcaattataagctagtagataagataacttctgaccaacatatcttcagtccagacaaaatagatatgttaacactggggaaaatgctcatgccaactataaaaggtcagaaaacagatcagttcttgaacaagagagagaattatttccatgggaacaatcttattgagtctttgtcagcagcgttagcatgtcattggtgtgggatattaacagagcaatgtatagaaaataatattttcaagaaagactggggtgacgggttcatatcggatcatgcttttatggacttcaaaatattcctatgtgtctttaaaactaaacttttatgtagttggggatcccaagggaaaaacattaaagatgaagatatagtagatgaatcgatagataaactgttaaggattgataatactttttggagaatgttcagcaaggttatgtttgaatcaaaggttaagaaaaggataatgttatatgatgtaaaatttctatcattagtaggttatatagggtttaagaattggtttatagaacagttgagatcagctgagttgcatgaggtaccttggattgtcaatgccgaaggtgatctggttgagatcaagtcaattaaaatctatttgcaactgatagagcagagtttatttttaagaataactgttttgaactatacagatatggcacatgctctcacaagattaatcagaaagaagttgatgtgtgataatgcactattaacttcaattccatccccaatggttaacttaactcaagttattgatcctacagaacaattagcttatttccctaagataacatttgaaaggctaaaaaattatgacactagttcaaattatgctaaaggaaagctaacaaggaattacatgatactgttgccatggcaacatgttaatagatataactttgtctttagttctactggatgtaaagttagtctaaaaacatgcattggaaaacttatgaaagatctaaaccctaaagttctgtactttattggagaaggggcaggaaattggatggccagaacagcatgtgaatatcctgacatcaaatttgtatacagaagtttaaaagatgaccttgatcatcattatcctttggaataccagagagtgataggagaattaagcaggataatagatagtggtgaagggctttcaatggaaacaacagatgcaactcaaaaaactcattgggatttgatacacagagtaagcaaagatgctttattaataactttatgtgatgcagaatttaaggacagagatgatttttttaagatggtaattctatggaggaaacatgtattatcatgcagaatttgcactacctatgggacagacctctatttattcgcaaagtatcatgctaaagactgcaatataaaattacctttttttgtgagatcagttgccacctttattatgcaaggtagtaaactgtcaggctcggaatgctacatactcttaacactaggccaccacaacaatttaccttgtcatggagaaatacaaaattctaagatgaaaatagcagcgtgtaatgatttttatgctgcaaaaaaacttgacaataaatcaattgaagccaactgtaaatcacttttatcagggctaagaataccgataaataagaaggaattaaatagacagagaaggttattaacactacaaagcaaccattcttctgtagcaacagttggaggtagcaaggtcatagagtctaaatggttaacaaacaaggcaaacacaataattgattggttagaacatattttaaattctccaaaaggtgaattaaattatgatttttttgaagcattagaaaatacttaccctaatatgattaaactaatagataatctagggaatgcagagattaaaaaactgatcaaagtaactggatatatgcttgtaagtaaaaaatgaaaaatgataaaaatgataaaataggtgacaacttcatactattccaaagtaatcatttgattatgcaattatgtaatagttaattaaaaactaaaaatcaaaagttaaaaactaataactgtcattaagtttattaaaaataagaaattataattggatgtatacggtttttttgccgt

SEQ ID NO: 3 - DNA, 12473 bp, metapneumovirus
gcgaaaaaaacgcgtataaattagattacaaaaaaatatgggacaagtgaaaatgtctcttcaagggattcacctgagtgatctatcatacaagcatgctatattaaaagagtctcagtacacaataaaaagagatgtgggtacaacaactgcagtgacaccctcatcattgcaacaagaaataacgctgttgtgtggagaaattctgtatgctaaacatgctgattacaaatatgctgcagaaataggaatacaatatattagcacagctttaggatcagagagagtgcagcagattctgaggaactcaggcagtgaagtccaagtggtcttaaccagaacgtactctctggggaaagttaaaaacaataaaggagaagatttacagatgttagacatacacggggtagagaagagctgggtagaagagatagacaaagaagcaaggaaaacaatggcaaccttgcttaaggaatcatcaggtaatatcccacaaaatcagaggccctcagcaccagacacacccataatcttattatgtgtaggtgcattaatatttactaagctagcatcaaccatagaagtgggactagagaccacagtcagaagggctaaccgtgtactaagtgatgcactcaagagataccctagaatggacatcccaaaaattgccagatccttctatgacttatttgaacaaaaagtgtatcacagaagtttgttcattgagtatggcaaagcattaggctcatcatctacaggcagcaaagcagaaagtctatttgttaatatattcatgcaagcttatggagccggtcaaacaatgctaaggtggggggtcattgccaggtcatccaacaatataatgttaggacatgtatctgtccaagctgagttaaaacaggtcacagaagtctatgacttggtgcgagaaatgggccctgaatctggacttctacatttaaggcaaagcccaaaagctggactgttatcactagccaactgtcccaactttgcaagtgttgttctcggaaatgcctcaggcttaggcataatcggtatgtatcgtgggagagtaccaaacacagaattattttcagcagcagaaagttatgccaaaagtttgaaagagagcaataaaatcaatttctcttcattaggacttacagatgaagagaaagaggctgcagaacatttcttaaatgtgagtgacgacagtcaaaatgattatgagtaattaaaaaagtgggacaagtcaaaatgtctttccctgaaggaaaagatattcttttcatgggtaatgaagcagcaaaattagcagaagctttccagaaatcattaaggaaaccaagtcataaaagatctcaatctattataggagaaaaagtgaacactgtatcagaaacattggaattacctactatcagtagacctgcaaaaccaaccatactgtcagaaccaaagttagcatggactgataaaggtggggcaatcaaaactgaaataaagcaagcaatcaaagtcatggatcctattgaggaagaagagtctactgagaagaaggtgctgccctccagtgatgggaaaacccctgcagaaaagaaactgaaaccatcaactaacaccaaaaagaaagtttcgtttacaccaaatgaaccaggaaaatatacaaagttggaaaaagatgctctagatttgctctcagataatgaagaagaagatgcagaatcttcaatcttaacctttgaagaaagagatacttcatcgttaagcattgaggccagattggaatcaatagaggagaaattaagcatgatattagggctattaagaacactcaacattgctacagcaggacccacagcagcaagagatgggatcagagatgcaatgattggcgtaagagaggaattaatagcagacataataaaggaagccaaagggaaagcagcagaaatgatggaagaggaaatgagtcaacgatcaaaaataggaaacggtagtgtaaaactaacagagaaagcaaaagagcttaacaaaattgttgaagatgaaagcacaagtggagaatctgaagaagaagaagaaccaaaagacatacaagacaatagtcaagaagatgacatttaccagttaattatgtagtttaataaaaataaacaatgggacaagtaaaaatggagtcctacctagtagacacttatcaaggcattccttacacagcagctgttcaagttgatctaatagaaaaggacctgttacctgcaagcctaacaatatggttccctttgtttcaggccaacacaccaccagcagtgctgctcgatcagttgaaaaccctaacaataaccactctgtatgctgcatcacaaaatggtccaatactcaaagtgaatgcatcagcccaaggtgcagcaatgtctgtacttcccaaaaaatttgaagtcaatgcgactgtagcactcgatgaatatagcaaattggaatttgacaaactcacagtctgtgaagtaaaaacagtttacttaacaaccatgaaaccatacgggatggtatcaaaatttgtgagctcagccaaatcagttggcaaaaaaacacatgatctaatcgcactgtgtgattttatggatctagaaaagaacacacctgttacaataccagcattcatcaaatcagtttcaatcaaagagagtgagtcagctactgttgaagctgctataagcagtgaagcagaccaagctctaacacaggccaaaattgcaccttatgcgggattgattatgatcatgactatgaacaatcccaaaggcatattcaaaaagcttggagctgggactcaagttatagtagaactaggagcatatgtccaggctgaaagcataagtaaaatatgcaagacttggagccatcaagggacaagatatgtgttgaagtccagataacagccaagcaccttggccaagagctactaactctatctcatagattataaagtcaccattctagttatataaaaatcaagttagaacaagaattaaatcaatcaagaatgggacaaataaaaatgtcttggaaagtggtgatcattttttcattgttaataacacctcaacacggtcttaaagagagctatttagaagagtcatgtagcactataactgaaggatatctcagtgttctgaggacaggttggtataccaacgtttttacactggaggtaggtgatgtagagaaccttacatgtgctgatggacctagcttaataaaaacagaattagacctgaccaaaagtgcactaagagaactcagaacagtttctgctgatcaactggcaagagaggagcaaattgagaatcccagacaatctagatttgttctaggagcaatagcactcggtgttgcaacagcagctgcagttacagcaggtgttgcaattgccaaaaccatccggcttgaaagtgaagtaacagcaattaagaatgccctcaaaaagaccaatgaagcagtatctacattggggaatggagttcgagtgttggcaactgcagtgagggagctggaagattttgtgagcaagaatctaacacgtgcaatcaacaaaaacaagtgcgacattgctgacctgaaaatggccgttagcttcagtcaattcaacagaaggtttctaaatgttgtgcggcaattttcagacaatgctggaataacaccagcaatatccttggacttaatgacagatgctgaactagccagagctgtttccaacatgccaacatctgcaggacaaataaaactgatgttggagaaccgtgcaatggtaagaagaaaggggttcggaatcctgataggagtttacggaagctccgtaatttacatggtgcaactgccaatctttggagttatagacacgccttgctggatagtaaaagcggccccttcttgctcagaaaaaaagggaaactatgcttgccttttaagagaagatcaaggatggtattgtcagaatgcagggtcaactgtttactacccaaatgaaaaagactgcgaaacaagaggagaccatgtcttttgcgacacagcagcaggaatcaatgttgctgagcagtcaaaggagtgcaacatcaacatatccactactaattacccatgcaaagttagcacaggaagacaccctatcagtatggttgcactgtctcctcttggggctttggttgcttgctacaagggagtgagctgttccattggcagcaacagagtagggatcatcaagcaactgaacaaaggctgctcttatataaccaaccaagacgcagacacagtgacaatagacaacactgtataccagctaagcaaagttgagggcgaacagcatgttataaaaggaaggccagtgtcaagcagctttgatccagtcaaatttcctgaagatcaattcaatgttgcacttgaccaagttttcgaaagcattgagaacagtcaggccttggtggatcaatcaaacagaatcctaagcagtgcagagaaaggaaacactggcttcatcattgtaataattctaattgctgtccttggctctaccatgatcctagtgagtgtttttatcataataaagaaaacaaagaaacccacaggagcacctccagagctgagtggtgtcacaaacaatggcttcataccacataattagttaattaaaaataaagtaaattaaattaaaataaaataaaattaaaattaaaataaaataaaaataaaaatttgggacaaatcataatgtctcgcaaggctccatgcaaatatgaagtgcggggcaaatgcaatagaggaagtgagtgcaagtttaaccacaattactggagttggccagatagatacttactaataagatcaaattatttattaaatcaacttttaaggaacactgatagagctgatggcttatcaataatatcaggagcaggcagagaagataggacacaagattttgtcctaggttccaccaatgtggttcaaggttatattgatgataaccaaagcataacaaaagctgcagcctgttacagtctacataatataatcaaacaactacaagaagttgaagttaggcaggctagagataacaaaccatctgacagcaaacatgtggcacttcacaacttagtcctatcttatatggagatgagcaaaattcctgcatctttaatcaacaatctcaaaagactgccgagagagaaactgaaaaaattagcaaagcttataattgacttatcagcaggtgctgaaaatgactcttcatatgccttgcaagacagtgaaagcactaatcaagtgcagtgagcatggtcctgttttcattactatagaggttgattacatgatatggactcataaggacttaaaagaagctttatctaatgggatagtgaagtctcatactaacatttacaattgttatttagaaaacatagaaattatatatgtcaaggcttacttaagttagtaaaaacacatcagagtgggataaatgacaatgataacattagatgtcattaaaagtgatgggtcttcaaaaacatgtactcacctcaaaaaattaattaaagaccactctggtaaagtgcttattgtacttaagttaatattagctttactaacatttctcacagtgacaatcaccatcaattatataaaagtagaaaacaatctgcaaatatgtcagtcaaaaactgaatcagacaaaaaggactcatcatcaaataccacatcagtcacaaccaagactactctaaatcatgatataacacagtattttaaaagtttgattcaaaggtatacaaactctgcaataaacagagacacatgctggaaaataagcagaaatcaatgcacaaacataacaacatacaaatttttatgttttaaatctgaagaaacaaaaaccaacaattgtgataaactgacagatttatgcagaaacaaaccaaaaccagctgttgaagtgtatcacatagtagaatgccattgtatatacacagttaaatggaagtgctatcattacccaatagatgaaacccaatcctaaataacactagattaggatccatccaagtctgttagttcaacaatttagttatttaaaaatattttgaaaacaagtaagtttctatgatacttcataataataagtaataattaattgcttaatcatcatcacaacattattcgaaaccataactattcaatttaagaagtaaaaacaataatatgagacaaataacaatggatcctcttaatgaatccactgttaatgtctatcttcccgactcatatcttaaaggagtgatttcttttagtgagactaatgcaattggttcatgtctcttaaaaagaccttacctaaaaaatgacaacactgcaaaagttgccatagagaatcctgttatcgagcatgttagactcaaaaatgcaatcaattctaagatgaaaatatcagattacaggatagtagagccagtaaacatgcaacatgaaattatgaagaatgtacacagttgtgagctcacattattaaaacagtttttaacaaggagtaaaaatattagcactcttaaattaaatatgatatgtgattggctgcagttaaagtctacatcagatgatacctcaatcttaagttttatagatgtagaatttatacctagctgggtaagcaattggtttagtaattggtacaatctcaacaagttgattctggaattcaggaaagaagaagtaataagaactggttcaatcttgtgtaggtcattgggtaaattagtttttgttgtatcatcatacggatgtatagtcaagagcaacaaaagcaaaagagtgagcttcttcacatacaatcaactgttaacatggaaagatgtgatgttaagtagattcaatgcaaatttctgtatatgggtaagcaacagtctgaatgaaaatcaagaagggttagggttgagaagtaatctgcaaggcatattaactaataagctatatgaaactgtagattatatgcttagtttgtgttgcaatgaaggtttctcacttgtgaaagagtttgagggttttattatgagtgaaatccttaggattactgaacatgctcaattcagtactagatttagaaatactttattaaatggattaactgatcaattgacaaaattaaaaaataaaaacagactcagagttcatggtaccgtgttagaaaataatgattatccaatgtatgaagttgtacttaaattattaggagatactttgagatgtattaaattattaatcaataaaaacttagagaatgctgctgaattatactatatatttagaatattcggtcacccaatggtagatgaaagagatgcaatggatgctgtcaaattaaacaatgaaatcacaaaaatcctcaggttggagagcttgacagaactaagaggggcattcatattaaggattatcaaaggatttgtagacaacaacaaaagatggccgaaaattaaaaacttaaaagtgcttagtaaaagatggactatgtacttcaaagcaaaaagttaccctagtcaacttgaattaagtgaacaagattttttagagcttgctgcaatacagtttgaacaagagttttctgttcctgaaaaaaccaaccttgagatggtattaaatgataaagctatatcacctcctaaaagattaatttggtctgtgtacccaaaaaattacttacctgagacaataaaaaatcgatatctagaagagactttcaatgcaagtgatagtctcaaaacaagaagagtactagagtactatttgaaagataataaattcgaccaaaaagaacttaaaagttatgtggttaaacaagaatatttaaatgataaggatcatattgtctcgctaactggaaaagaaagagaattaagtgtaggtagaatgtttgctatgcaaccaggaaaacagcgacaaatacaaatattggctgaaaaattgttagctgataatattgtaccctttttcccagaaactttaacaaagtatggtgatctagatcttcagagaataatggaaatcaaatcagaactttcttctattaaaaccagaagaaatgatagttataataattacattgcaagagcatccatagtaacagatttaagtaagttcaaccaagcctttaggtatgaaactacagcgatctgtgcggatgtagcagatgaactacatggaacacaaagcctattctgttggttacatcttatcgttcctatgactacaatgatatgtgcctatagacatgcaccaccagaaacaaaaggtgaatatgatatagataagatagaagagcaaagtggtttatatagatatcatatgggtggtattgaaggatggtgtcaaaaactctggacaatggaagctatatctttattagatgttgtatctgtaaagacacgatgtcaaatgacatctttattaaacggtgacaaccaatcaatagatgtaagtaaaccagttaagttatctgagggtttagatgaagtgaaagcagattatagcttggctgtaaaaatgctaaaagaaataagagatgcatacagaaatataggccataaacttaaagaaggggaaacatatatatcaagagatcttcagtttataagtaaggtgattcaatctgaaggagtaatgcatcctacccctataaaaaagatcttaagagtgggaccatggataaacacaatattagatgacattaaaaccagtgcagagtcaatagggagtctatgtcaggaattagaatttaggggggaaagcataatagttagtctgatattaaggaatttttggctgtataatttatacatgcatgaatcaaagcaacaccccctagcagggaagcagttattcaaacaactaaataaaacattaacatcagtgcagagattttttgaaattaaaaaggaaaatgaagtagtagatctatggatgaacataccaatgcagtttggaggaggagatccagtagtcttctatagatctttctatagaaggacccctgattttttaactgaagcaatcagtcatgtagatattctgttaaaaatatcagccaacataagaaatgaagcgaaaataagtttcttcaaagccttactgtcaatagaaaaaaatgaacgtgctacactgacaacactaatgagagaccctcaagctgtgggctcagagcgacaagcaaaagtaacaagtgatatcaatagaacagcagttaccagcatcttaagtctttctccaaatcaacttttcagcgatagtgctatacactacagtagaaatgaagaagaggtcggaatcattgctgacaacataacacctgtttatcctcatggactgagagttttgtatgaatcattaccttttcataaagctgaaaaagttgtaaatatgatatcaggaacaaaatccataaccaacttattacagagaacatctgctattaatggtgaagatattgacagagctgtatccatgatgctggagaacctaggattattatctagaatattgtcagtagttgttgatagtatagaaattccaaccaaatctaatggtaggctgatatgttgtcagatatctagaaccctaagggagacatcatggaataatatggaaatagttggagtaacatcccctagcatcactacatgcatggatgtcatatatgcaactagctctcatttgaaagggataatcattgaaaagttcagcactgacagaactacaagaggtcaaagaggtccaaagagcccttgggtaggatcgagcacgcaagagaaaaaattagttcctgtttataacagacaaattctttcaaaacaacaaagagaacagctagaagcaattggaaaaatgagatgggtatataaagggacaccaggtttaagacgattactcaataagatttgtcttggaagtttaggcattagttacaaatgtgtaaaacctttattacctaggtttatgagtgtaaatttcctacacaggttatctgtcagtagtagacctatggaattcccagcatcagttccagcttatagaacaacaaattaccattttgacactagtcctattaatcaagcactaagtgaaagatttgggaatgaagatattaatttggtcttccaaaatgcaatcagctgtggaattagcataatgagtgtagtagaacaattaactggtaggagtccaaaacagttagttttaataccccaattagaagaaatagacattatgccaccaccagtgtttcaagggaaattcaattataagctagtagataagataacttctgaccaacatatcttcagtccagacaaaatagatatgttaacactggggaaaatgctcatgccaactataaaaggtcagaaaacagatcagttcttgaacaagagagagaattatttccatgggaacaatcttattgagtctttgtcagcagcgttagcatgtcattggtgtgggatattaacagagcaatgtatagaaaataatattttcaagaaagactggggtgacgggttcatatcggatcatgcttttatggacttcaaaatattcctatgtgtctttaaaactaaacttttatgtagttggggatcccaagggaaaaacattaaagatgaagatatagtagatgaatcgatagataaactgttaaggattgataatactttttggagaatgttcagcaaggttatgtttgaatcaaaggttaagaaaaggataatgttatatgatgtaaaatttctatcattagtaggttatatagggtttaagaattggtttatagaacagttgagatcagctgagttgcatgaggtaccttggattgtcaatgccgaaggtgatctggttgagatcaagtcaattaaaatctatttgcaactgatagagcagagtttatttttaagaataactgttttgaactatacagatatggcacatgctctcacaagattaatcagaaagaagttgatgtgtgataatgcactattaacttcaattccatccccaatggttaacttaactcaagttattgatcctacagaacaattagcttatttccctaagataacatttgaaaggctaaaaaattatgacactagttcaaattatgctaaaggaaagctaacaaggaattacatgatactgttgccatggcaacatgttaatagatataactttgtctttagttctactggatgtaaagttagtctaaaaacatgcattggaaaacttatgaaagatctaaaccctaaagttctgtactttattggagaaggggcaggaaattggatggccagaacagcatgtgaatatcctgacatcaaatttgtatacagaagtttaaaagatgaccttgatcatcattatcctttggaataccagagagtgataggagaattaagcaggataatagatagtggtgaagggctttcaatggaaacaacagatgcaactcaaaaaactcattgggatttgatacacagagtaagcaaagatgctttattaataactttatgtgatgcagaatttaaggacagagatgatttttttaagatggtaattctatggaggaaacatgtattatcatgcagaatttgcactacctatgggacagacctctatttattcgcaaagtatcatgctaaagactgcaatataaaattacctttttttgtgagatcagttgccacctttattatgcaaggtagtaaactgtcaggctcggaatgctacatactcttaacactaggccaccacaacaatttaccttgtcatggagaaatacaaaattctaagatgaaaatagcagcgtgtaatgatttttatgctgcaaaaaaacttgacaataaatcaattgaagccaactgtaaatcacttttatcagggctaagaataccgataaataagaaggaattaaatagacagagaaggttattaacactacaaagcaaccattcttctgtagcaacagttggaggtagcaaggtcatagagtctaaatggttaacaaacaaggcaaacacaataattgattggttagaacatattttaaattctccaaaaggtgaattaaattatgatttttttgaagcattagaaaatacttaccctaatatgattaaactaatagataatctagggaatgcagagattaaaaaactgatcaaagtaactggatatatgcttgtaagtaaaaaatgaaaaatgataaaaatgataaaataggtgacaacttcatactattccaaagtaatcatttgattatgcaattatgtaatagttaattaaaaactaaaaatcaaaagttaaaaactaataactgtcattaagtttattaaaaataagaaattataattggatgtatacggtttttttgccgt

SEQ ID NO: 4 - DNA, 14141 bp, Artificial Sequence
  Le gène de la GFP est inséré entre les positions 40 et 784
gcgaaaaaaacgcgtataaattagattacaaaaaaatatgggacaagtgaaaatggtgagcaagggcgaggagctgttcaccggggtggtgcccatcctggtcgagctggacggcgacgtaaacggccacaagttcagcgtgtccggcgagggcgagggcgatgccacctacggcaagctgaccctgaagttcatctgcaccaccggcaagctgcccgtgccctggcccaccctcgtgaccaccctgacctacggcgtgcagtgcttcagccgctaccccgaccacatgaagcagcacgacttcttcaagtccgccatgcccgaaggctacgtccaggagcgcaccatcttcttcaaggacgacggcaactacaagacccgcgccgaggtgaagttcgagggcgacaccctggtgaaccgcatcgagctgaagggcatcgacttcaaggaggacggcaacatcctggggcacaagctggagtacaactacaacagccacaacgtctatatcatggccgacaagcagaagaacggcatcaaggtgaacttcaagatccgccacaacatcgaggacggcagcgtgcagctcgccgaccactaccagcagaacacccccatcggcgacggccccgtgctgctgcccgacaaccactacctgagcacccagtccgccctgagcaaagaccccaacgagaagcgcgatcacatggtcctgctggagttcgtgaccgccgccgggatcactctcggcatggacgagctgtacaagtaagttaattaaaaagtgggacaagtgaaaatgtctcttcaagggattcacctgagtgatctatcatacaagcatgctatattaaaagagtctcagtacacaataaaaagagatgtgggtacaacaactgcagtgacaccctcatcattgcaacaagaaataacgctgttgtgtggagaaattctgtatgctaaacatgctgattacaaatatgctgcagaaataggaatacaatatattagcacagctttaggatcagagagagtgcagcagattctgaggaactcaggcagtgaagtccaagtggtcttaaccagaacgtactctctggggaaagttaaaaacaataaaggagaagatttacagatgttagacatacacggggtagagaagagctgggtagaagagatagacaaagaagcaaggaaaacaatggcaaccttgcttaaggaatcatcaggtaatatcccacaaaatcagaggccctcagcaccagacacacccataatcttattatgtgtaggtgcattaatatttactaagctagcatcaaccatagaagtgggactagagaccacagtcagaagggctaaccgtgtactaagtgatgcactcaagagataccctagaatggacatcccaaaaattgccagatccttctatgacttatttgaacaaaaagtgtatcacagaagtttgttcattgagtatggcaaagcattaggctcatcatctacaggcagcaaagcagaaagtctatttgttaatatattcatgcaagcttatggagccggtcaaacaatgctaaggtggggggtcattgccaggtcatccaacaatataatgttaggacatgtatctgtccaagctgagttaaaacaggtcacagaagtctatgacttggtgcgagaaatgggccctgaatctggacttctacatttaaggcaaagcccaaaagctggactgttatcactagccaactgtcccaactttgcaagtgttgttctcggaaatgcctcaggcttaggcataatcggtatgtatcgtgggagagtaccaaacacagaattattttcagcagcagaaagttatgccaaaagtttgaaagagagcaataaaatcaatttctcttcattaggacttacagatgaagagaaagaggctgcagaacatttcttaaatgtgagtgacgacagtcaaaatgattatgagtaattaaaaaagtgggacaagtcaaaatgtctttccctgaaggaaaagatattcttttcatgggtaatgaagcagcaaaattagcagaagctttccagaaatcattaaggaaaccaagtcataaaagatctcaatctattataggagaaaaagtgaacactgtatcagaaacattggaattacctactatcagtagacctgcaaaaccaaccatactgtcagaaccaaagttagcatggactgataaaggtggggcaatcaaaactgaaataaagcaagcaatcaaagtcatggatcctattgaggaagaagagtctactgagaagaaggtgctgccctccagtgatgggaaaacccctgcagaaaagaaactgaaaccatcaactaacaccaaaaagaaagtttcgtttacaccaaatgaaccaggaaaatatacaaagttggaaaaagatgctctagatttgctctcagataatgaagaagaagatgcagaatcttcaatcttaacctttgaagaaagagatacttcatcgttaagcattgaggccagattggaatcaatagaggagaaattaagcatgatattagggctattaagaacactcaacattgctacagcaggacccacagcagcaagagatgggatcagagatgcaatgattggcgtaagagaggaattaatagcagacataataaaggaagccaaagggaaagcagcagaaatgatggaagaggaaatgagtcaacgatcaaaaataggaaacggtagtgtaaaactaacagagaaagcaaaagagcttaacaaaattgttgaagatgaaagcacaagtggagaatctgaagaagaagaagaaccaaaagacatacaagacaatagtcaagaagatgacatttaccagttaattatgtagtttaataaaaataaacaatgggacaagtaaaaatggagtcctacctagtagacacttatcaaggcattccttacacagcagctgttcaagttgatctaatagaaaaggacctgttacctgcaagcctaacaatatggttccctttgtttcaggccaacacaccaccagcagtgctgctcgatcagttgaaaaccctaacaataaccactctgtatgctgcatcacaaaatggtccaatactcaaagtgaatgcatcagcccaaggtgcagcaatgtctgtacttcccaaaaaatttgaagtcaatgcgactgtagcactcgatgaatatagcaaattggaatttgacaaactcacagtctgtgaagtaaaaacagtttacttaacaaccatgaaaccatacgggatggtatcaaaatttgtgagctcagccaaatcagttggcaaaaaaacacatgatctaatcgcactgtgtgattttatggatctagaaaagaacacacctgttacaataccagcattcatcaaatcagtttcaatcaaagagagtgagtcagctactgttgaagctgctataagcagtgaagcagaccaagctctaacacaggccaaaattgcaccttatgcgggattgattatgatcatgactatgaacaatcccaaaggcatattcaaaaagcttggagctgggactcaagttatagtagaactaggagcatatgtccaggctgaaagcataagtaaaatatgcaagacttggagccatcaagggacaagatatgtgttgaagtccagataacagccaagcaccttggccaagagctactaactctatctcatagattataaagtcaccattctagttatataaaaatcaagttagaacaagaattaaatcaatcaagaatgggacaaataaaaatgtcttggaaagtggtgatcattttttcattgttaataacacctcaacacggtcttaaagagagctatttagaagagtcatgtagcactataactgaaggatatctcagtgttctgaggacaggttggtataccaacgtttttacactggaggtaggtgatgtagagaaccttacatgtgctgatggacctagcttaataaaaacagaattagacctgaccaaaagtgcactaagagaactcagaacagtttctgctgatcaactggcaagagaggagcaaattgagaatcccagacaatctagatttgttctaggagcaatagcactcggtgttgcaacagcagctgcagttacagcaggtgttgcaattgccaaaaccatccggcttgaaagtgaagtaacagcaattaagaatgccctcaaaaagaccaatgaagcagtatctacattggggaatggagttcgagtgttggcaactgcagtgagggagctggaagattttgtgagcaagaatctaacacgtgcaatcaacaaaaacaagtgcgacattgctgacctgaaaatggccgttagcttcagtcaattcaacagaaggtttctaaatgttgtgcggcaattttcagacaatgctggaataacaccagcaatatccttggacttaatgacagatgctgaactagccagagctgtttccaacatgccaacatctgcaggacaaataaaactgatgttggagaaccgtgcaatggtaagaagaaaggggttcggaatcctgataggagtttacggaagctccgtaatttacatggtgcaactgccaatctttggagttatagacacgccttgctggatagtaaaagcggccccttcttgctcagaaaaaaagggaaactatgcttgccttttaagagaagatcaaggatggtattgtcagaatgcagggtcaactgtttactacccaaatgaaaaagactgcgaaacaagaggagaccatgtcttttgcgacacagcagcaggaatcaatgttgctgagcagtcaaaggagtgcaacatcaacatatccactactaattacccatgcaaagttagcacaggaagacaccctatcagtatggttgcactgtctcctcttggggctttggttgcttgctacaagggagtgagctgttccattggcagcaacagagtagggatcatcaagcaactgaacaaaggctgctcttatataaccaaccaagacgcagacacagtgacaatagacaacactgtataccagctaagcaaagttgagggcgaacagcatgttataaaaggaaggccagtgtcaagcagctttgatccagtcaaatttcctgaagatcaattcaatgttgcacttgaccaagttttcgaaagcattgagaacagtcaggccttggtggatcaatcaaacagaatcctaagcagtgcagagaaaggaaacactggcttcatcattgtaataattctaattgctgtccttggctctaccatgatcctagtgagtgtttttatcataataaagaaaacaaagaaacccacaggagcacctccagagctgagtggtgtcacaaacaatggcttcataccacataattagttaattaaaaataaagtaaattaaattaaaataaaataaaattaaaattaaaataaaataaaaataaaaatttgggacaaatcataatgtctcgcaaggctccatgcaaatatgaagtgcggggcaaatgcaatagaggaagtgagtgcaagtttaaccacaattactggagttggccagatagatacttactaataagatcaaattatttattaaatcaacttttaaggaacactgatagagctgatggcttatcaataatatcaggagcaggcagagaagataggacacaagattttgtcctaggttccaccaatgtggttcaaggttatattgatgataaccaaagcataacaaaagctgcagcctgttacagtctacataatataatcaaacaactacaagaagttgaagttaggcaggctagagataacaaaccatctgacagcaaacatgtggcacttcacaacttagtcctatcttatatggagatgagcaaaattcctgcatctttaatcaacaatctcaaaagactgccgagagagaaactgaaaaaattagcaaagcttataattgacttatcagcaggtgctgaaaatgactcttcatatgccttgcaagacagtgaaagcactaatcaagtgcagtgagcatggtcctgttttcattactatagaggttgattacatgatatggactcataaggacttaaaagaagctttatctaatgggatagtgaagtctcatactaacatttacaattgttatttagaaaacatagaaattatatatgtcaaggcttacttaagttagtaaaaacacatcagagtgggataaatgacaatgataacattagatgtcattaaaagtgatgggtcttcaaaaacatgtactcacctcaaaaaattaattaaagaccactctggtaaagtgcttattgtacttaagttaatattagctttactaacatttctcacagtgacaatcaccatcaattatataaaagtagaaaacaatctgcaaatatgtcagtcaaaaactgaatcagacaaaaaggactcatcatcaaataccacatcagtcacaaccaagactactctaaatcatgatataacacagtattttaaaagtttgattcaaaggtatacaaactctgcaataaacagagacacatgctggaaaataagcagaaatcaatgcacaaacataacaacatacaaatttttatgttttaaatctgaagaaacaaaaaccaacaattgtgataaactgacagatttatgcagaaacaaaccaaaaccagctgttgaagtgtatcacatagtagaatgccattgtatatacacagttaaatggaagtgctatcattacccaatagatgaaacccaatcctaaataacactagattaggatccatccaagtctgttagttcaacaatttagttatttaaaaatattttgaaaacaagtaagtttctatgatacttcataataataagtaataattaattgcttaatcatcatcacaacattattcgaaaccataactattcaatttaagaagtaaaaacaataatatgggacaagtagttatggaggtgaaagtggagaacattcgaacaatagatatgctcaaagcaagagtgaaaaatcgtgtggcacgcagcaaatgctttaaaaatgcctctttgatcctaataggaataactacattgagtatagccctcaatatctatctaatcataaactatacaatgcaagaaaacacatccgaatcagaacatcacaccagctcatcacccatggaatccagcagggaaactccaacagtccctatggacaactcagacaccaatccaggctcacagtatccaactcaacagtccacagaaggctccacactctactttgcagcctcagcaagctcaccagagacagaaccaacatcaacaccagacacaacaagccgcccgcccttcgtcgacacacacacaacactaccaagtgcaagcagaacaaggacaagtccggcagtccacacaaaaaacaatccaaggacaagccccagaacacattccccaccatgggcaatgacaaggacggtccgtggaaccaccactctccgcacaagcagcacaagaaaaagaccgtccacagcatcagtccaacctgacagcagcgcaacaacccacaaacacgaagaagcaagcccagtgagcccgcaaacatctgcgagcacagcaagaccacaaaggaagggcatggaggccagcacatcaacaacatacaaccaaactagttaacaaaaaatacaaaataactctaagataaaccatatagacaccaacaattgagaagccaaaaggcaattcacaatctctccaaaaaggcaacaacaccatattagctccgcttaaatctccctggaaaaaacactcgcccatataccaactataccacaaccatcccaagaaaaaaagctgggtaaaacaacacccaagagacaaataacaatggatcctcttaatgaatccactgttaatgtctatcttcccgactcatatcttaaaggagtgatttcttttagtgagactaatgcaattggttcatgtctcttaaaaagaccttacctaaaaaatgacaacactgcaaaagttgccatagagaatcctgttatcgagcatgttagactcaaaaatgcaatcaattctaagatgaaaatatcagattacaggatagtagagccagtaaacatgcaacatgaaattatgaagaatgtacacagttgtgagctcacattattaaaacagtttttaacaaggagtaaaaatattagcactcttaaattaaatatgatatgtgattggctgcagttaaagtctacatcagatgatacctcaatcttaagttttatagatgtagaatttatacctagctgggtaagcaattggtttagtaattggtacaatctcaacaagttgattctggaattcaggaaagaagaagtaataagaactggttcaatcttgtgtaggtcattgggtaaattagtttttgttgtatcatcatacggatgtatagtcaagagcaacaaaagcaaaagagtgagcttcttcacatacaatcaactgttaacatggaaagatgtgatgttaagtagattcaatgcaaatttctgtatatgggtaagcaacagtctgaatgaaaatcaagaagggttagggttgagaagtaatctgcaaggcatattaactaataagctatatgaaactgtagattatatgcttagtttgtgttgcaatgaaggtttctcacttgtgaaagagtttgagggttttattatgagtgaaatccttaggattactgaacatgctcaattcagtactagatttagaaatactttattaaatggattaactgatcaattgacaaaattaaaaaataaaaacagactcagagttcatggtaccgtgttagaaaataatgattatccaatgtatgaagttgtacttaaattattaggagatactttgagatgtattaaattattaatcaataaaaacttagagaatgctgctgaattatactatatatttagaatattcggtcacccaatggtagatgaaagagatgcaatggatgctgtcaaattaaacaatgaaatcacaaaaatcctcaggttggagagcttgacagaactaagaggggcattcatattaaggattatcaaaggatttgtagacaacaacaaaagatggccgaaaattaaaaacttaaaagtgcttagtaaaagatggactatgtacttcaaagcaaaaagttaccctagtcaacttgaattaagtgaacaagattttttagagcttgctgcaatacagtttgaacaagagttttctgttcctgaaaaaaccaaccttgagatggtattaaatgataaagctatatcacctcctaaaagattaatttggtctgtgtacccaaaaaattacttacctgagacaataaaaaatcgatatctagaagagactttcaatgcaagtgatagtctcaaaacaagaagagtactagagtactatttgaaagataataaattcgaccaaaaagaacttaaaagttatgtggttaaacaagaatatttaaatgataaggatcatattgtctcgctaactggaaaagaaagagaattaagtgtaggtagaatgtttgctatgcaaccaggaaaacagcgacaaatacaaatattggctgaaaaattgttagctgataatattgtaccctttttcccagaaactttaacaaagtatggtgatctagatcttcagagaataatggaaatcaaatcagaactttcttctattaaaaccagaagaaatgatagttataataattacattgcaagagcatccatagtaacagatttaagtaagttcaaccaagcctttaggtatgaaactacagcgatctgtgcggatgtagcagatgaactacatggaacacaaagcctattctgttggttacatcttatcgttcctatgactacaatgatatgtgcctatagacatgcaccaccagaaacaaaaggtgaatatgatatagataagatagaagagcaaagtggtttatatagatatcatatgggtggtattgaaggatggtgtcaaaaactctggacaatggaagctatatctttattagatgttgtatctgtaaagacacgatgtcaaatgacatctttattaaacggtgacaaccaatcaatagatgtaagtaaaccagttaagttatctgagggtttagatgaagtgaaagcagattatagcttggctgtaaaaatgctaaaagaaataagagatgcatacagaaatataggccataaacttaaagaaggggaaacatatatatcaagagatcttcagtttataagtaaggtgattcaatctgaaggagtaatgcatcctacccctataaaaaagatcttaagagtgggaccatggataaacacaatattagatgacattaaaaccagtgcagagtcaatagggagtctatgtcaggaattagaatttaggggggaaagcataatagttagtctgatattaaggaatttttggctgtataatttatacatgcatgaatcaaagcaacaccccctagcagggaagcagttattcaaacaactaaataaaacattaacatcagtgcagagattttttgaaattaaaaaggaaaatgaagtagtagatctatggatgaacataccaatgcagtttggaggaggagatccagtagtcttctatagatctttctatagaaggacccctgattttttaactgaagcaatcagtcatgtagatattctgttaaaaatatcagccaacataagaaatgaagcgaaaataagtttcttcaaagccttactgtcaatagaaaaaaatgaacgtgctacactgacaacactaatgagagaccctcaagctgtgggctcagagcgacaagcaaaagtaacaagtgatatcaatagaacagcagttaccagcatcttaagtctttctccaaatcaacttttcagcgatagtgctatacactacagtagaaatgaagaagaggtcggaatcattgctgacaacataacacctgtttatcctcatggactgagagttttgtatgaatcattaccttttcataaagctgaaaaagttgtaaatatgatatcaggaacaaaatccataaccaacttattacagagaacatctgctattaatggtgaagatattgacagagctgtatccatgatgctggagaacctaggattattatctagaatattgtcagtagttgttgatagtatagaaattccaaccaaatctaatggtaggctgatatgttgtcagatatctagaaccctaagggagacatcatggaataatatggaaatagttggagtaacatcccctagcatcactacatgcatggatgtcatatatgcaactagctctcatttgaaagggataatcattgaaaagttcagcactgacagaactacaagaggtcaaagaggtccaaagagcccttgggtaggatcgagcacgcaagagaaaaaattagttcctgtttataacagacaaattctttcaaaacaacaaagagaacagctagaagcaattggaaaaatgagatgggtatataaagggacaccaggtttaagacgattactcaataagatttgtcttggaagtttaggcattagttacaaatgtgtaaaacctttattacctaggtttatgagtgtaaatttcctacacaggttatctgtcagtagtagacctatggaattcccagcatcagttccagcttatagaacaacaaattaccattttgacactagtcctattaatcaagcactaagtgaaagatttgggaatgaagatattaatttggtcttccaaaatgcaatcagctgtggaattagcataatgagtgtagtagaacaattaactggtaggagtccaaaacagttagttttaataccccaattagaagaaatagacattatgccaccaccagtgtttcaagggaaattcaattataagctagtagataagataacttctgaccaacatatcttcagtccagacaaaatagatatgttaacactggggaaaatgctcatgccaactataaaaggtcagaaaacagatcagttcttgaacaagagagagaattatttccatgggaacaatcttattgagtctttgtcagcagcgttagcatgtcattggtgtgggatattaacagagcaatgtatagaaaataatattttcaagaaagactggggtgacgggttcatatcggatcatgcttttatggacttcaaaatattcctatgtgtctttaaaactaaacttttatgtagttggggatcccaagggaaaaacattaaagatgaagatatagtagatgaatcgatagataaactgttaaggattgataatactttttggagaatgttcagcaaggttatgtttgaatcaaaggttaagaaaaggataatgttatatgatgtaaaatttctatcattagtaggttatatagggtttaagaattggtttatagaacagttgagatcagctgagttgcatgaggtaccttggattgtcaatgccgaaggtgatctggttgagatcaagtcaattaaaatctatttgcaactgatagagcagagtttatttttaagaataactgttttgaactatacagatatggcacatgctctcacaagattaatcagaaagaagttgatgtgtgataatgcactattaacttcaattccatccccaatggttaacttaactcaagttattgatcctacagaacaattagcttatttccctaagataacatttgaaaggctaaaaaattatgacactagttcaaattatgctaaaggaaagctaacaaggaattacatgatactgttgccatggcaacatgttaatagatataactttgtctttagttctactggatgtaaagttagtctaaaaacatgcattggaaaacttatgaaagatctaaaccctaaagttctgtactttattggagaaggggcaggaaattggatggccagaacagcatgtgaatatcctgacatcaaatttgtatacagaagtttaaaagatgaccttgatcatcattatcctttggaataccagagagtgataggagaattaagcaggataatagatagtggtgaagggctttcaatggaaacaacagatgcaactcaaaaaactcattgggatttgatacacagagtaagcaaagatgctttattaataactttatgtgatgcagaatttaaggacagagatgatttttttaagatggtaattctatggaggaaacatgtattatcatgcagaatttgcactacctatgggacagacctctatttattcgcaaagtatcatgctaaagactgcaatataaaattacctttttttgtgagatcagttgccacctttattatgcaaggtagtaaactgtcaggctcggaatgctacatactcttaacactaggccaccacaacaatttaccttgtcatggagaaatacaaaattctaagatgaaaatagcagcgtgtaatgatttttatgctgcaaaaaaacttgacaataaatcaattgaagccaactgtaaatcacttttatcagggctaagaataccgataaataagaaggaattaaatagacagagaaggttattaacactacaaagcaaccattcttctgtagcaacagttggaggtagcaaggtcatagagtctaaatggttaacaaacaaggcaaacacaataattgattggttagaacatattttaaattctccaaaaggtgaattaaattatgatttttttgaagcattagaaaatacttaccctaatatgattaaactaatagataatctagggaatgcagagattaaaaaactgatcaaagtaactggatatatgcttgtaagtaaaaaatgaaaaatgataaaaatgataaaataggtgacaacttcatactattccaaagtaatcatttgattatgcaattatgtaatagttaattaaaaactaaaaatcaaaagttaaaaactaataactgtcattaagtttattaaaaataagaaattataattggatgtatacggtttttttgccgt

SEQ ID NO: 5 - DNA, 13392 bp, Artificial Sequence
  Le gène de la GFP est inséré entre les positions 40 et 784
gcgaaaaaaacgcgtataaattagattacaaaaaaatatgggacaagtgaaaatggtgagcaagggcgaggagctgttcaccggggtggtgcccatcctggtcgagctggacggcgacgtaaacggccacaagttcagcgtgtccggcgagggcgagggcgatgccacctacggcaagctgaccctgaagttcatctgcaccaccggcaagctgcccgtgccctggcccaccctcgtgaccaccctgacctacggcgtgcagtgcttcagccgctaccccgaccacatgaagcagcacgacttcttcaagtccgccatgcccgaaggctacgtccaggagcgcaccatcttcttcaaggacgacggcaactacaagacccgcgccgaggtgaagttcgagggcgacaccctggtgaaccgcatcgagctgaagggcatcgacttcaaggaggacggcaacatcctggggcacaagctggagtacaactacaacagccacaacgtctatatcatggccgacaagcagaagaacggcatcaaggtgaacttcaagatccgccacaacatcgaggacggcagcgtgcagctcgccgaccactaccagcagaacacccccatcggcgacggccccgtgctgctgcccgacaaccactacctgagcacccagtccgccctgagcaaagaccccaacgagaagcgcgatcacatggtcctgctggagttcgtgaccgccgccgggatcactctcggcatggacgagctgtacaagtaagttaattaaaaagtgggacaagtgaaaatgtctcttcaagggattcacctgagtgatctatcatacaagcatgctatattaaaagagtctcagtacacaataaaaagagatgtgggtacaacaactgcagtgacaccctcatcattgcaacaagaaataacgctgttgtgtggagaaattctgtatgctaaacatgctgattacaaatatgctgcagaaataggaatacaatatattagcacagctttaggatcagagagagtgcagcagattctgaggaactcaggcagtgaagtccaagtggtcttaaccagaacgtactctctggggaaagttaaaaacaataaaggagaagatttacagatgttagacatacacggggtagagaagagctgggtagaagagatagacaaagaagcaaggaaaacaatggcaaccttgcttaaggaatcatcaggtaatatcccacaaaatcagaggccctcagcaccagacacacccataatcttattatgtgtaggtgcattaatatttactaagctagcatcaaccatagaagtgggactagagaccacagtcagaagggctaaccgtgtactaagtgatgcactcaagagataccctagaatggacatcccaaaaattgccagatccttctatgacttatttgaacaaaaagtgtatcacagaagtttgttcattgagtatggcaaagcattaggctcatcatctacaggcagcaaagcagaaagtctatttgttaatatattcatgcaagcttatggagccggtcaaacaatgctaaggtggggggtcattgccaggtcatccaacaatataatgttaggacatgtatctgtccaagctgagttaaaacaggtcacagaagtctatgacttggtgcgagaaatgggccctgaatctggacttctacatttaaggcaaagcccaaaagctggactgttatcactagccaactgtcccaactttgcaagtgttgttctcggaaatgcctcaggcttaggcataatcggtatgtatcgtgggagagtaccaaacacagaattattttcagcagcagaaagttatgccaaaagtttgaaagagagcaataaaatcaatttctcttcattaggacttacagatgaagagaaagaggctgcagaacatttcttaaatgtgagtgacgacagtcaaaatgattatgagtaattaaaaaagtgggacaagtcaaaatgtctttccctgaaggaaaagatattcttttcatgggtaatgaagcagcaaaattagcagaagctttccagaaatcattaaggaaaccaagtcataaaagatctcaatctattataggagaaaaagtgaacactgtatcagaaacattggaattacctactatcagtagacctgcaaaaccaaccatactgtcagaaccaaagttagcatggactgataaaggtggggcaatcaaaactgaaataaagcaagcaatcaaagtcatggatcctattgaggaagaagagtctactgagaagaaggtgctgccctccagtgatgggaaaacccctgcagaaaagaaactgaaaccatcaactaacaccaaaaagaaagtttcgtttacaccaaatgaaccaggaaaatatacaaagttggaaaaagatgctctagatttgctctcagataatgaagaagaagatgcagaatcttcaatcttaacctttgaagaaagagatacttcatcgttaagcattgaggccagattggaatcaatagaggagaaattaagcatgatattagggctattaagaacactcaacattgctacagcaggacccacagcagcaagagatgggatcagagatgcaatgattggcgtaagagaggaattaatagcagacataataaaggaagccaaagggaaagcagcagaaatgatggaagaggaaatgagtcaacgatcaaaaataggaaacggtagtgtaaaactaacagagaaagcaaaagagcttaacaaaattgttgaagatgaaagcacaagtggagaatctgaagaagaagaagaaccaaaagacatacaagacaatagtcaagaagatgacatttaccagttaattatgtagtttaataaaaataaacaatgggacaagtaaaaatggagtcctacctagtagacacttatcaaggcattccttacacagcagctgttcaagttgatctaatagaaaaggacctgttacctgcaagcctaacaatatggttccctttgtttcaggccaacacaccaccagcagtgctgctcgatcagttgaaaaccctaacaataaccactctgtatgctgcatcacaaaatggtccaatactcaaagtgaatgcatcagcccaaggtgcagcaatgtctgtacttcccaaaaaatttgaagtcaatgcgactgtagcactcgatgaatatagcaaattggaatttgacaaactcacagtctgtgaagtaaaaacagtttacttaacaaccatgaaaccatacgggatggtatcaaaatttgtgagctcagccaaatcagttggcaaaaaaacacatgatctaatcgcactgtgtgattttatggatctagaaaagaacacacctgttacaataccagcattcatcaaatcagtttcaatcaaagagagtgagtcagctactgttgaagctgctataagcagtgaagcagaccaagctctaacacaggccaaaattgcaccttatgcgggattgattatgatcatgactatgaacaatcccaaaggcatattcaaaaagcttggagctgggactcaagttatagtagaactaggagcatatgtccaggctgaaagcataagtaaaatatgcaagacttggagccatcaagggacaagatatgtgttgaagtccagataacagccaagcaccttggccaagagctactaactctatctcatagattataaagtcaccattctagttatataaaaatcaagttagaacaagaattaaatcaatcaagaatgggacaaataaaaatgtcttggaaagtggtgatcattttttcattgttaataacacctcaacacggtcttaaagagagctatttagaagagtcatgtagcactataactgaaggatatctcagtgttctgaggacaggttggtataccaacgtttttacactggaggtaggtgatgtagagaaccttacatgtgctgatggacctagcttaataaaaacagaattagacctgaccaaaagtgcactaagagaactcagaacagtttctgctgatcaactggcaagagaggagcaaattgagaatcccagacaatctagatttgttctaggagcaatagcactcggtgttgcaacagcagctgcagttacagcaggtgttgcaattgccaaaaccatccggcttgaaagtgaagtaacagcaattaagaatgccctcaaaaagaccaatgaagcagtatctacattggggaatggagttcgagtgttggcaactgcagtgagggagctggaagattttgtgagcaagaatctaacacgtgcaatcaacaaaaacaagtgcgacattgctgacctgaaaatggccgttagcttcagtcaattcaacagaaggtttctaaatgttgtgcggcaattttcagacaatgctggaataacaccagcaatatccttggacttaatgacagatgctgaactagccagagctgtttccaacatgccaacatctgcaggacaaataaaactgatgttggagaaccgtgcaatggtaagaagaaaggggttcggaatcctgataggagtttacggaagctccgtaatttacatggtgcaactgccaatctttggagttatagacacgccttgctggatagtaaaagcggccccttcttgctcagaaaaaaagggaaactatgcttgccttttaagagaagatcaaggatggtattgtcagaatgcagggtcaactgtttactacccaaatgaaaaagactgcgaaacaagaggagaccatgtcttttgcgacacagcagcaggaatcaatgttgctgagcagtcaaaggagtgcaacatcaacatatccactactaattacccatgcaaagttagcacaggaagacaccctatcagtatggttgcactgtctcctcttggggctttggttgcttgctacaagggagtgagctgttccattggcagcaacagagtagggatcatcaagcaactgaacaaaggctgctcttatataaccaaccaagacgcagacacagtgacaatagacaacactgtataccagctaagcaaagttgagggcgaacagcatgttataaaaggaaggccagtgtcaagcagctttgatccagtcaaatttcctgaagatcaattcaatgttgcacttgaccaagttttcgaaagcattgagaacagtcaggccttggtggatcaatcaaacagaatcctaagcagtgcagagaaaggaaacactggcttcatcattgtaataattctaattgctgtccttggctctaccatgatcctagtgagtgtttttatcataataaagaaaacaaagaaacccacaggagcacctccagagctgagtggtgtcacaaacaatggcttcataccacataattagttaattaaaaataaagtaaattaaattaaaataaaataaaattaaaattaaaataaaataaaaataaaaatttgggacaaatcataatgtctcgcaaggctccatgcaaatatgaagtgcggggcaaatgcaatagaggaagtgagtgcaagtttaaccacaattactggagttggccagatagatacttactaataagatcaaattatttattaaatcaacttttaaggaacactgatagagctgatggcttatcaataatatcaggagcaggcagagaagataggacacaagattttgtcctaggttccaccaatgtggttcaaggttatattgatgataaccaaagcataacaaaagctgcagcctgttacagtctacataatataatcaaacaactacaagaagttgaagttaggcaggctagagataacaaaccatctgacagcaaacatgtggcacttcacaacttagtcctatcttatatggagatgagcaaaattcctgcatctttaatcaacaatctcaaaagactgccgagagagaaactgaaaaaattagcaaagcttataattgacttatcagcaggtgctgaaaatgactcttcatatgccttgcaagacagtgaaagcactaatcaagtgcagtgagcatggtcctgttttcattactatagaggttgattacatgatatggactcataaggacttaaaagaagctttatctaatgggatagtgaagtctcatactaacatttacaattgttatttagaaaacatagaaattatatatgtcaaggcttacttaagttagtaaaaacacatcagagtgggacaagtagttatggaggtgaaagtggagaacattcgaacaatagatatgctcaaagcaagagtgaaaaatcgtgtggcacgcagcaaatgctttaaaaatgcctctttgatcctaataggaataactacattgagtatagccctcaatatctatctaatcataaactatacaatgcaagaaaacacatccgaatcagaacatcacaccagctcatcacccatggaatccagcagggaaactccaacagtccctatggacaactcagacaccaatccaggctcacagtatccaactcaacagtccacagaaggctccacactctactttgcagcctcagcaagctcaccagagacagaaccaacatcaacaccagacacaacaagccgcccgcccttcgtcgacacacacacaacactaccaagtgcaagcagaacaaggacaagtccggcagtccacacaaaaaacaatccaaggacaagccccagaacacattccccaccatgggcaatgacaaggacggtccgtggaaccaccactctccgcacaagcagcacaagaaaaagaccgtccacagcatcagtccaacctgacagcagcgcaacaacccacaaacacgaagaagcaagcccagtgagcccgcaaacatctgcgagcacagcaagaccacaaaggaagggcatggaggccagcacatcaacaacatacaaccaaactagttaacaaaaaatacaaaataactctaagataaaccatatagacaccaacaattgagaagccaaaaggcaattcacaatctctccaaaaaggcaacaacaccatattagctccgcttaaatctccctggaaaaaacactcgcccatataccaactataccacaaccatcccaagaaaaaaagctgggtaaaacaacacccaagagacaaataacaatggatcctcttaatgaatccactgttaatgtctatcttcccgactcatatcttaaaggagtgatttcttttagtgagactaatgcaattggttcatgtctcttaaaaagaccttacctaaaaaatgacaacactgcaaaagttgccatagagaatcctgttatcgagcatgttagactcaaaaatgcaatcaattctaagatgaaaatatcagattacaggatagtagagccagtaaacatgcaacatgaaattatgaagaatgtacacagttgtgagctcacattattaaaacagtttttaacaaggagtaaaaatattagcactcttaaattaaatatgatatgtgattggctgcagttaaagtctacatcagatgatacctcaatcttaagttttatagatgtagaatttatacctagctgggtaagcaattggtttagtaattggtacaatctcaacaagttgattctggaattcaggaaagaagaagtaataagaactggttcaatcttgtgtaggtcattgggtaaattagtttttgttgtatcatcatacggatgtatagtcaagagcaacaaaagcaaaagagtgagcttcttcacatacaatcaactgttaacatggaaagatgtgatgttaagtagattcaatgcaaatttctgtatatgggtaagcaacagtctgaatgaaaatcaagaagggttagggttgagaagtaatctgcaaggcatattaactaataagctatatgaaactgtagattatatgcttagtttgtgttgcaatgaaggtttctcacttgtgaaagagtttgagggttttattatgagtgaaatccttaggattactgaacatgctcaattcagtactagatttagaaatactttattaaatggattaactgatcaattgacaaaattaaaaaataaaaacagactcagagttcatggtaccgtgttagaaaataatgattatccaatgtatgaagttgtacttaaattattaggagatactttgagatgtattaaattattaatcaataaaaacttagagaatgctgctgaattatactatatatttagaatattcggtcacccaatggtagatgaaagagatgcaatggatgctgtcaaattaaacaatgaaatcacaaaaatcctcaggttggagagcttgacagaactaagaggggcattcatattaaggattatcaaaggatttgtagacaacaacaaaagatggccgaaaattaaaaacttaaaagtgcttagtaaaagatggactatgtacttcaaagcaaaaagttaccctagtcaacttgaattaagtgaacaagattttttagagcttgctgcaatacagtttgaacaagagttttctgttcctgaaaaaaccaaccttgagatggtattaaatgataaagctatatcacctcctaaaagattaatttggtctgtgtacccaaaaaattacttacctgagacaataaaaaatcgatatctagaagagactttcaatgcaagtgatagtctcaaaacaagaagagtactagagtactatttgaaagataataaattcgaccaaaaagaacttaaaagttatgtggttaaacaagaatatttaaatgataaggatcatattgtctcgctaactggaaaagaaagagaattaagtgtaggtagaatgtttgctatgcaaccaggaaaacagcgacaaatacaaatattggctgaaaaattgttagctgataatattgtaccctttttcccagaaactttaacaaagtatggtgatctagatcttcagagaataatggaaatcaaatcagaactttcttctattaaaaccagaagaaatgatagttataataattacattgcaagagcatccatagtaacagatttaagtaagttcaaccaagcctttaggtatgaaactacagcgatctgtgcggatgtagcagatgaactacatggaacacaaagcctattctgttggttacatcttatcgttcctatgactacaatgatatgtgcctatagacatgcaccaccagaaacaaaaggtgaatatgatatagataagatagaagagcaaagtggtttatatagatatcatatgggtggtattgaaggatggtgtcaaaaactctggacaatggaagctatatctttattagatgttgtatctgtaaagacacgatgtcaaatgacatctttattaaacggtgacaaccaatcaatagatgtaagtaaaccagttaagttatctgagggtttagatgaagtgaaagcagattatagcttggctgtaaaaatgctaaaagaaataagagatgcatacagaaatataggccataaacttaaagaaggggaaacatatatatcaagagatcttcagtttataagtaaggtgattcaatctgaaggagtaatgcatcctacccctataaaaaagatcttaagagtgggaccatggataaacacaatattagatgacattaaaaccagtgcagagtcaatagggagtctatgtcaggaattagaatttaggggggaaagcataatagttagtctgatattaaggaatttttggctgtataatttatacatgcatgaatcaaagcaacaccccctagcagggaagcagttattcaaacaactaaataaaacattaacatcagtgcagagattttttgaaattaaaaaggaaaatgaagtagtagatctatggatgaacataccaatgcagtttggaggaggagatccagtagtcttctatagatctttctatagaaggacccctgattttttaactgaagcaatcagtcatgtagatattctgttaaaaatatcagccaacataagaaatgaagcgaaaataagtttcttcaaagccttactgtcaatagaaaaaaatgaacgtgctacactgacaacactaatgagagaccctcaagctgtgggctcagagcgacaagcaaaagtaacaagtgatatcaatagaacagcagttaccagcatcttaagtctttctccaaatcaacttttcagcgatagtgctatacactacagtagaaatgaagaagaggtcggaatcattgctgacaacataacacctgtttatcctcatggactgagagttttgtatgaatcattaccttttcataaagctgaaaaagttgtaaatatgatatcaggaacaaaatccataaccaacttattacagagaacatctgctattaatggtgaagatattgacagagctgtatccatgatgctggagaacctaggattattatctagaatattgtcagtagttgttgatagtatagaaattccaaccaaatctaatggtaggctgatatgttgtcagatatctagaaccctaagggagacatcatggaataatatggaaatagttggagtaacatcccctagcatcactacatgcatggatgtcatatatgcaactagctctcatttgaaagggataatcattgaaaagttcagcactgacagaactacaagaggtcaaagaggtccaaagagcccttgggtaggatcgagcacgcaagagaaaaaattagttcctgtttataacagacaaattctttcaaaacaacaaagagaacagctagaagcaattggaaaaatgagatgggtatataaagggacaccaggtttaagacgattactcaataagatttgtcttggaagtttaggcattagttacaaatgtgtaaaacctttattacctaggtttatgagtgtaaatttcctacacaggttatctgtcagtagtagacctatggaattcccagcatcagttccagcttatagaacaacaaattaccattttgacactagtcctattaatcaagcactaagtgaaagatttgggaatgaagatattaatttggtcttccaaaatgcaatcagctgtggaattagcataatgagtgtagtagaacaattaactggtaggagtccaaaacagttagttttaataccccaattagaagaaatagacattatgccaccaccagtgtttcaagggaaattcaattataagctagtagataagataacttctgaccaacatatcttcagtccagacaaaatagatatgttaacactggggaaaatgctcatgccaactataaaaggtcagaaaacagatcagttcttgaacaagagagagaattatttccatgggaacaatcttattgagtctttgtcagcagcgttagcatgtcattggtgtgggatattaacagagcaatgtatagaaaataatattttcaagaaagactggggtgacgggttcatatcggatcatgcttttatggacttcaaaatattcctatgtgtctttaaaactaaacttttatgtagttggggatcccaagggaaaaacattaaagatgaagatatagtagatgaatcgatagataaactgttaaggattgataatactttttggagaatgttcagcaaggttatgtttgaatcaaaggttaagaaaaggataatgttatatgatgtaaaatttctatcattagtaggttatatagggtttaagaattggtttatagaacagttgagatcagctgagttgcatgaggtaccttggattgtcaatgccgaaggtgatctggttgagatcaagtcaattaaaatctatttgcaactgatagagcagagtttatttttaagaataactgttttgaactatacagatatggcacatgctctcacaagattaatcagaaagaagttgatgtgtgataatgcactattaacttcaattccatccccaatggttaacttaactcaagttattgatcctacagaacaattagcttatttccctaagataacatttgaaaggctaaaaaattatgacactagttcaaattatgctaaaggaaagctaacaaggaattacatgatactgttgccatggcaacatgttaatagatataactttgtctttagttctactggatgtaaagttagtctaaaaacatgcattggaaaacttatgaaagatctaaaccctaaagttctgtactttattggagaaggggcaggaaattggatggccagaacagcatgtgaatatcctgacatcaaatttgtatacagaagtttaaaagatgaccttgatcatcattatcctttggaataccagagagtgataggagaattaagcaggataatagatagtggtgaagggctttcaatggaaacaacagatgcaactcaaaaaactcattgggatttgatacacagagtaagcaaagatgctttattaataactttatgtgatgcagaatttaaggacagagatgatttttttaagatggtaattctatggaggaaacatgtattatcatgcagaatttgcactacctatgggacagacctctatttattcgcaaagtatcatgctaaagactgcaatataaaattacctttttttgtgagatcagttgccacctttattatgcaaggtagtaaactgtcaggctcggaatgctacatactcttaacactaggccaccacaacaatttaccttgtcatggagaaatacaaaattctaagatgaaaatagcagcgtgtaatgatttttatgctgcaaaaaaacttgacaataaatcaattgaagccaactgtaaatcacttttatcagggctaagaataccgataaataagaaggaattaaatagacagagaaggttattaacactacaaagcaaccattcttctgtagcaacagttggaggtagcaaggtcatagagtctaaatggttaacaaacaaggcaaacacaataattgattggttagaacatattttaaattctccaaaaggtgaattaaattatgatttttttgaagcattagaaaatacttaccctaatatgattaaactaatagataatctagggaatgcagagattaaaaaactgatcaaagtaactggatatatgcttgtaagtaaaaaatgaaaaatgataaaaatgataaaataggtgacaacttcatactattccaaagtaatcatttgattatgcaattatgtaatagttaattaaaaactaaaaatcaaaagttaaaaactaataactgtcattaagtttattaaaaataagaaattataattggatgtatacggtttttttgccgt

SEQ ID NO: 6 - DNA, 13220 bp, Artificial Sequence
  Le gène de la GFP est inséré entre les positions 40 et 784
gcgaaaaaaacgcgtataaattagattacaaaaaaatatgggacaagtgaaaatggtgagcaagggcgaggagctgttcaccggggtggtgcccatcctggtcgagctggacggcgacgtaaacggccacaagttcagcgtgtccggcgagggcgagggcgatgccacctacggcaagctgaccctgaagttcatctgcaccaccggcaagctgcccgtgccctggcccaccctcgtgaccaccctgacctacggcgtgcagtgcttcagccgctaccccgaccacatgaagcagcacgacttcttcaagtccgccatgcccgaaggctacgtccaggagcgcaccatcttcttcaaggacgacggcaactacaagacccgcgccgaggtgaagttcgagggcgacaccctggtgaaccgcatcgagctgaagggcatcgacttcaaggaggacggcaacatcctggggcacaagctggagtacaactacaacagccacaacgtctatatcatggccgacaagcagaagaacggcatcaaggtgaacttcaagatccgccacaacatcgaggacggcagcgtgcagctcgccgaccactaccagcagaacacccccatcggcgacggccccgtgctgctgcccgacaaccactacctgagcacccagtccgccctgagcaaagaccccaacgagaagcgcgatcacatggtcctgctggagttcgtgaccgccgccgggatcactctcggcatggacgagctgtacaagtaagttaattaaaaagtgggacaagtgaaaatgtctcttcaagggattcacctgagtgatctatcatacaagcatgctatattaaaagagtctcagtacacaataaaaagagatgtgggtacaacaactgcagtgacaccctcatcattgcaacaagaaataacgctgttgtgtggagaaattctgtatgctaaacatgctgattacaaatatgctgcagaaataggaatacaatatattagcacagctttaggatcagagagagtgcagcagattctgaggaactcaggcagtgaagtccaagtggtcttaaccagaacgtactctctggggaaagttaaaaacaataaaggagaagatttacagatgttagacatacacggggtagagaagagctgggtagaagagatagacaaagaagcaaggaaaacaatggcaaccttgcttaaggaatcatcaggtaatatcccacaaaatcagaggccctcagcaccagacacacccataatcttattatgtgtaggtgcattaatatttactaagctagcatcaaccatagaagtgggactagagaccacagtcagaagggctaaccgtgtactaagtgatgcactcaagagataccctagaatggacatcccaaaaattgccagatccttctatgacttatttgaacaaaaagtgtatcacagaagtttgttcattgagtatggcaaagcattaggctcatcatctacaggcagcaaagcagaaagtctatttgttaatatattcatgcaagcttatggagccggtcaaacaatgctaaggtggggggtcattgccaggtcatccaacaatataatgttaggacatgtatctgtccaagctgagttaaaacaggtcacagaagtctatgacttggtgcgagaaatgggccctgaatctggacttctacatttaaggcaaagcccaaaagctggactgttatcactagccaactgtcccaactttgcaagtgttgttctcggaaatgcctcaggcttaggcataatcggtatgtatcgtgggagagtaccaaacacagaattattttcagcagcagaaagttatgccaaaagtttgaaagagagcaataaaatcaatttctcttcattaggacttacagatgaagagaaagaggctgcagaacatttcttaaatgtgagtgacgacagtcaaaatgattatgagtaattaaaaaagtgggacaagtcaaaatgtctttccctgaaggaaaagatattcttttcatgggtaatgaagcagcaaaattagcagaagctttccagaaatcattaaggaaaccaagtcataaaagatctcaatctattataggagaaaaagtgaacactgtatcagaaacattggaattacctactatcagtagacctgcaaaaccaaccatactgtcagaaccaaagttagcatggactgataaaggtggggcaatcaaaactgaaataaagcaagcaatcaaagtcatggatcctattgaggaagaagagtctactgagaagaaggtgctgccctccagtgatgggaaaacccctgcagaaaagaaactgaaaccatcaactaacaccaaaaagaaagtttcgtttacaccaaatgaaccaggaaaatatacaaagttggaaaaagatgctctagatttgctctcagataatgaagaagaagatgcagaatcttcaatcttaacctttgaagaaagagatacttcatcgttaagcattgaggccagattggaatcaatagaggagaaattaagcatgatattagggctattaagaacactcaacattgctacagcaggacccacagcagcaagagatgggatcagagatgcaatgattggcgtaagagaggaattaatagcagacataataaaggaagccaaagggaaagcagcagaaatgatggaagaggaaatgagtcaacgatcaaaaataggaaacggtagtgtaaaactaacagagaaagcaaaagagcttaacaaaattgttgaagatgaaagcacaagtggagaatctgaagaagaagaagaaccaaaagacatacaagacaatagtcaagaagatgacatttaccagttaattatgtagtttaataaaaataaacaatgggacaagtaaaaatggagtcctacctagtagacacttatcaaggcattccttacacagcagctgttcaagttgatctaatagaaaaggacctgttacctgcaagcctaacaatatggttccctttgtttcaggccaacacaccaccagcagtgctgctcgatcagttgaaaaccctaacaataaccactctgtatgctgcatcacaaaatggtccaatactcaaagtgaatgcatcagcccaaggtgcagcaatgtctgtacttcccaaaaaatttgaagtcaatgcgactgtagcactcgatgaatatagcaaattggaatttgacaaactcacagtctgtgaagtaaaaacagtttacttaacaaccatgaaaccatacgggatggtatcaaaatttgtgagctcagccaaatcagttggcaaaaaaacacatgatctaatcgcactgtgtgattttatggatctagaaaagaacacacctgttacaataccagcattcatcaaatcagtttcaatcaaagagagtgagtcagctactgttgaagctgctataagcagtgaagcagaccaagctctaacacaggccaaaattgcaccttatgcgggattgattatgatcatgactatgaacaatcccaaaggcatattcaaaaagcttggagctgggactcaagttatagtagaactaggagcatatgtccaggctgaaagcataagtaaaatatgcaagacttggagccatcaagggacaagatatgtgttgaagtccagataacagccaagcaccttggccaagagctactaactctatctcatagattataaagtcaccattctagttatataaaaatcaagttagaacaagaattaaatcaatcaagaatgggacaaataaaaatgtcttggaaagtggtgatcattttttcattgttaataacacctcaacacggtcttaaagagagctatttagaagagtcatgtagcactataactgaaggatatctcagtgttctgaggacaggttggtataccaacgtttttacactggaggtaggtgatgtagagaaccttacatgtgctgatggacctagcttaataaaaacagaattagacctgaccaaaagtgcactaagagaactcagaacagtttctgctgatcaactggcaagagaggagcaaattgagaatcccagacaatctagatttgttctaggagcaatagcactcggtgttgcaacagcagctgcagttacagcaggtgttgcaattgccaaaaccatccggcttgaaagtgaagtaacagcaattaagaatgccctcaaaaagaccaatgaagcagtatctacattggggaatggagttcgagtgttggcaactgcagtgagggagctggaagattttgtgagcaagaatctaacacgtgcaatcaacaaaaacaagtgcgacattgctgacctgaaaatggccgttagcttcagtcaattcaacagaaggtttctaaatgttgtgcggcaattttcagacaatgctggaataacaccagcaatatccttggacttaatgacagatgctgaactagccagagctgtttccaacatgccaacatctgcaggacaaataaaactgatgttggagaaccgtgcaatggtaagaagaaaggggttcggaatcctgataggagtttacggaagctccgtaatttacatggtgcaactgccaatctttggagttatagacacgccttgctggatagtaaaagcggccccttcttgctcagaaaaaaagggaaactatgcttgccttttaagagaagatcaaggatggtattgtcagaatgcagggtcaactgtttactacccaaatgaaaaagactgcgaaacaagaggagaccatgtcttttgcgacacagcagcaggaatcaatgttgctgagcagtcaaaggagtgcaacatcaacatatccactactaattacccatgcaaagttagcacaggaagacaccctatcagtatggttgcactgtctcctcttggggctttggttgcttgctacaagggagtgagctgttccattggcagcaacagagtagggatcatcaagcaactgaacaaaggctgctcttatataaccaaccaagacgcagacacagtgacaatagacaacactgtataccagctaagcaaagttgagggcgaacagcatgttataaaaggaaggccagtgtcaagcagctttgatccagtcaaatttcctgaagatcaattcaatgttgcacttgaccaagttttcgaaagcattgagaacagtcaggccttggtggatcaatcaaacagaatcctaagcagtgcagagaaaggaaacactggcttcatcattgtaataattctaattgctgtccttggctctaccatgatcctagtgagtgtttttatcataataaagaaaacaaagaaacccacaggagcacctccagagctgagtggtgtcacaaacaatggcttcataccacataattagttaattaaaaataaagtaaattaaattaaaataaaataaaattaaaattaaaataaaataaaaataaaaatttgggacaaatcataatgtctcgcaaggctccatgcaaatatgaagtgcggggcaaatgcaatagaggaagtgagtgcaagtttaaccacaattactggagttggccagatagatacttactaataagatcaaattatttattaaatcaacttttaaggaacactgatagagctgatggcttatcaataatatcaggagcaggcagagaagataggacacaagattttgtcctaggttccaccaatgtggttcaaggttatattgatgataaccaaagcataacaaaagctgcagcctgttacagtctacataatataatcaaacaactacaagaagttgaagttaggcaggctagagataacaaaccatctgacagcaaacatgtggcacttcacaacttagtcctatcttatatggagatgagcaaaattcctgcatctttaatcaacaatctcaaaagactgccgagagagaaactgaaaaaattagcaaagcttataattgacttatcagcaggtgctgaaaatgactcttcatatgccttgcaagacagtgaaagcactaatcaagtgcagtgagcatggtcctgttttcattactatagaggttgattacatgatatggactcataaggacttaaaagaagctttatctaatgggatagtgaagtctcatactaacatttacaattgttatttagaaaacatagaaattatatatgtcaaggcttacttaagttagtaaaaacacatcagagtgggataaatgacaatgataacattagatgtcattaaaagtgatgggtcttcaaaaacatgtactcacctcaaaaaattaattaaagaccactctggtaaagtgcttattgtacttaagttaatattagctttactaacatttctcacagtgacaatcaccatcaattatataaaagtagaaaacaatctgcaaatatgtcagtcaaaaactgaatcagacaaaaaggactcatcatcaaataccacatcagtcacaaccaagactactctaaatcatgatataacacagtattttaaaagtttgattcaaaggtatacaaactctgcaataaacagagacacatgctggaaaataagcagaaatcaatgcacaaacataacaacatacaaatttttatgttttaaatctgaagaaacaaaaaccaacaattgtgataaactgacagatttatgcagaaacaaaccaaaaccagctgttgaagtgtatcacatagtagaatgccattgtatatacacagttaaatggaagtgctatcattacccaatagatgaaacccaatcctaaataacactagattaggatccatccaagtctgttagttcaacaatttagttatttaaaaatattttgaaaacaagtaagtttctatgatacttcataataataagtaataattaattgcttaatcatcatcacaacattattcgaaaccataactattcaatttaagaagtaaaaacaataatatgagacaaataacaatggatcctcttaatgaatccactgttaatgtctatcttcccgactcatatcttaaaggagtgatttcttttagtgagactaatgcaattggttcatgtctcttaaaaagaccttacctaaaaaatgacaacactgcaaaagttgccatagagaatcctgttatcgagcatgttagactcaaaaatgcaatcaattctaagatgaaaatatcagattacaggatagtagagccagtaaacatgcaacatgaaattatgaagaatgtacacagttgtgagctcacattattaaaacagtttttaacaaggagtaaaaatattagcactcttaaattaaatatgatatgtgattggctgcagttaaagtctacatcagatgatacctcaatcttaagttttatagatgtagaatttatacctagctgggtaagcaattggtttagtaattggtacaatctcaacaagttgattctggaattcaggaaagaagaagtaataagaactggttcaatcttgtgtaggtcattgggtaaattagtttttgttgtatcatcatacggatgtatagtcaagagcaacaaaagcaaaagagtgagcttcttcacatacaatcaactgttaacatggaaagatgtgatgttaagtagattcaatgcaaatttctgtatatgggtaagcaacagtctgaatgaaaatcaagaagggttagggttgagaagtaatctgcaaggcatattaactaataagctatatgaaactgtagattatatgcttagtttgtgttgcaatgaaggtttctcacttgtgaaagagtttgagggttttattatgagtgaaatccttaggattactgaacatgctcaattcagtactagatttagaaatactttattaaatggattaactgatcaattgacaaaattaaaaaataaaaacagactcagagttcatggtaccgtgttagaaaataatgattatccaatgtatgaagttgtacttaaattattaggagatactttgagatgtattaaattattaatcaataaaaacttagagaatgctgctgaattatactatatatttagaatattcggtcacccaatggtagatgaaagagatgcaatggatgctgtcaaattaaacaatgaaatcacaaaaatcctcaggttggagagcttgacagaactaagaggggcattcatattaaggattatcaaaggatttgtagacaacaacaaaagatggccgaaaattaaaaacttaaaagtgcttagtaaaagatggactatgtacttcaaagcaaaaagttaccctagtcaacttgaattaagtgaacaagattttttagagcttgctgcaatacagtttgaacaagagttttctgttcctgaaaaaaccaaccttgagatggtattaaatgataaagctatatcacctcctaaaagattaatttggtctgtgtacccaaaaaattacttacctgagacaataaaaaatcgatatctagaagagactttcaatgcaagtgatagtctcaaaacaagaagagtactagagtactatttgaaagataataaattcgaccaaaaagaacttaaaagttatgtggttaaacaagaatatttaaatgataaggatcatattgtctcgctaactggaaaagaaagagaattaagtgtaggtagaatgtttgctatgcaaccaggaaaacagcgacaaatacaaatattggctgaaaaattgttagctgataatattgtaccctttttcccagaaactttaacaaagtatggtgatctagatcttcagagaataatggaaatcaaatcagaactttcttctattaaaaccagaagaaatgatagttataataattacattgcaagagcatccatagtaacagatttaagtaagttcaaccaagcctttaggtatgaaactacagcgatctgtgcggatgtagcagatgaactacatggaacacaaagcctattctgttggttacatcttatcgttcctatgactacaatgatatgtgcctatagacatgcaccaccagaaacaaaaggtgaatatgatatagataagatagaagagcaaagtggtttatatagatatcatatgggtggtattgaaggatggtgtcaaaaactctggacaatggaagctatatctttattagatgttgtatctgtaaagacacgatgtcaaatgacatctttattaaacggtgacaaccaatcaatagatgtaagtaaaccagttaagttatctgagggtttagatgaagtgaaagcagattatagcttggctgtaaaaatgctaaaagaaataagagatgcatacagaaatataggccataaacttaaagaaggggaaacatatatatcaagagatcttcagtttataagtaaggtgattcaatctgaaggagtaatgcatcctacccctataaaaaagatcttaagagtgggaccatggataaacacaatattagatgacattaaaaccagtgcagagtcaatagggagtctatgtcaggaattagaatttaggggggaaagcataatagttagtctgatattaaggaatttttggctgtataatttatacatgcatgaatcaaagcaacaccccctagcagggaagcagttattcaaacaactaaataaaacattaacatcagtgcagagattttttgaaattaaaaaggaaaatgaagtagtagatctatggatgaacataccaatgcagtttggaggaggagatccagtagtcttctatagatctttctatagaaggacccctgattttttaactgaagcaatcagtcatgtagatattctgttaaaaatatcagccaacataagaaatgaagcgaaaataagtttcttcaaagccttactgtcaatagaaaaaaatgaacgtgctacactgacaacactaatgagagaccctcaagctgtgggctcagagcgacaagcaaaagtaacaagtgatatcaatagaacagcagttaccagcatcttaagtctttctccaaatcaacttttcagcgatagtgctatacactacagtagaaatgaagaagaggtcggaatcattgctgacaacataacacctgtttatcctcatggactgagagttttgtatgaatcattaccttttcataaagctgaaaaagttgtaaatatgatatcaggaacaaaatccataaccaacttattacagagaacatctgctattaatggtgaagatattgacagagctgtatccatgatgctggagaacctaggattattatctagaatattgtcagtagttgttgatagtatagaaattccaaccaaatctaatggtaggctgatatgttgtcagatatctagaaccctaagggagacatcatggaataatatggaaatagttggagtaacatcccctagcatcactacatgcatggatgtcatatatgcaactagctctcatttgaaagggataatcattgaaaagttcagcactgacagaactacaagaggtcaaagaggtccaaagagcccttgggtaggatcgagcacgcaagagaaaaaattagttcctgtttataacagacaaattctttcaaaacaacaaagagaacagctagaagcaattggaaaaatgagatgggtatataaagggacaccaggtttaagacgattactcaataagatttgtcttggaagtttaggcattagttacaaatgtgtaaaacctttattacctaggtttatgagtgtaaatttcctacacaggttatctgtcagtagtagacctatggaattcccagcatcagttccagcttatagaacaacaaattaccattttgacactagtcctattaatcaagcactaagtgaaagatttgggaatgaagatattaatttggtcttccaaaatgcaatcagctgtggaattagcataatgagtgtagtagaacaattaactggtaggagtccaaaacagttagttttaataccccaattagaagaaatagacattatgccaccaccagtgtttcaagggaaattcaattataagctagtagataagataacttctgaccaacatatcttcagtccagacaaaatagatatgttaacactggggaaaatgctcatgccaactataaaaggtcagaaaacagatcagttcttgaacaagagagagaattatttccatgggaacaatcttattgagtctttgtcagcagcgttagcatgtcattggtgtgggatattaacagagcaatgtatagaaaataatattttcaagaaagactggggtgacgggttcatatcggatcatgcttttatggacttcaaaatattcctatgtgtctttaaaactaaacttttatgtagttggggatcccaagggaaaaacattaaagatgaagatatagtagatgaatcgatagataaactgttaaggattgataatactttttggagaatgttcagcaaggttatgtttgaatcaaaggttaagaaaaggataatgttatatgatgtaaaatttctatcattagtaggttatatagggtttaagaattggtttatagaacagttgagatcagctgagttgcatgaggtaccttggattgtcaatgccgaaggtgatctggttgagatcaagtcaattaaaatctatttgcaactgatagagcagagtttatttttaagaataactgttttgaactatacagatatggcacatgctctcacaagattaatcagaaagaagttgatgtgtgataatgcactattaacttcaattccatccccaatggttaacttaactcaagttattgatcctacagaacaattagcttatttccctaagataacatttgaaaggctaaaaaattatgacactagttcaaattatgctaaaggaaagctaacaaggaattacatgatactgttgccatggcaacatgttaatagatataactttgtctttagttctactggatgtaaagttagtctaaaaacatgcattggaaaacttatgaaagatctaaaccctaaagttctgtactttattggagaaggggcaggaaattggatggccagaacagcatgtgaatatcctgacatcaaatttgtatacagaagtttaaaagatgaccttgatcatcattatcctttggaataccagagagtgataggagaattaagcaggataatagatagtggtgaagggctttcaatggaaacaacagatgcaactcaaaaaactcattgggatttgatacacagagtaagcaaagatgctttattaataactttatgtgatgcagaatttaaggacagagatgatttttttaagatggtaattctatggaggaaacatgtattatcatgcagaatttgcactacctatgggacagacctctatttattcgcaaagtatcatgctaaagactgcaatataaaattacctttttttgtgagatcagttgccacctttattatgcaaggtagtaaactgtcaggctcggaatgctacatactcttaacactaggccaccacaacaatttaccttgtcatggagaaatacaaaattctaagatgaaaatagcagcgtgtaatgatttttatgctgcaaaaaaacttgacaataaatcaattgaagccaactgtaaatcacttttatcagggctaagaataccgataaataagaaggaattaaatagacagagaaggttattaacactacaaagcaaccattcttctgtagcaacagttggaggtagcaaggtcatagagtctaaatggttaacaaacaaggcaaacacaataattgattggttagaacatattttaaattctccaaaaggtgaattaaattatgatttttttgaagcattagaaaatacttaccctaatatgattaaactaatagataatctagggaatgcagagattaaaaaactgatcaaagtaactggatatatgcttgtaagtaaaaaatgaaaaatgataaaaatgataaaataggtgacaacttcatactattccaaagtaatcatttgattatgcaattatgtaatagttaattaaaaactaaaaatcaaaagttaaaaactaataactgtcattaagtttattaaaaataagaaattataattggatgtatacggtttttttgccgt

SEQ ID NO: 7 - DNA, 13280 bp, metapneumovirus
acgcgaaaaaaacgcgtataaattaaattccaaacaaaacgggacaaataaaaatgtctcttcaagggattcacctaagtgatctgtcatataaacatgctatattaaaagagtctcaatacacaataaaaagagatgtaggcaccacaactgcagtgacaccttcatcattgcagcaagagataacacttttgtgtggagagattctttacactaaacatactgattacaaatatgctgcagagatagggatacaatatatttgcacggctctaggatcagaaagagtacaacagattttaagaaattcaggcagtgaagttcaggtggttctaaccaagacatactctttagggaaaggtaaaaatagtaaaggggaagagttgcaaatgttagatatacatggagtggaaaagagttgggtagaagaaatagacaaagaggcaagaaaaacaatggtgactttgctaaaggaatcatcaggtaacatcccacaaaaccagaggccttcagcaccagacacaccaataattttattatgtgtaggtgctttaatattcactaaactagcatcaacaatagaagttggactagagactacagttagaagagctaacagagtgctaagtgatgcgctcaaaagataccctagggtagatataccgaagattgctagatctttctatgaactatttgagcagaaagtgtattacaggagtctattcattgagtatgggaaagctttaggctcatcttcaacaggaagcaaagcagaaagtttgtttgtaaatatatttatgcaagcttatggagccggtcaaacaatgctaaggtggggtgtcattgccagatcatctaacaacataatgctaggacatgtgtctgtgcaagctgaattgaagcaagttacagaggtttatgatttggtgagagaaatgggtcctgaatctgggcttttacatctaagacaaagtccaaaggcaggactgttatcgttggccaattgccccgattttgctagtgttgttcttggtaatgcttcaggtctaggtataatcggaatgtacagaggaagagtgccaaacacagagctattttctgcagcagaaagttatgccagaagcttaaaagaaagcaacaaaatcaacttctcctcattagggctcacagacgaagaaaaagaagctgcagaacacttcttaaacatgagtgatgacaatcaagatgattatgagtaattaaaaaactgggacaagtcaaaatgtcattccctgaaggaaaagatatcctgttcatgggtaatgaagcagcaaaaatagcagaagctttccagaaatcactaaaaagatcaggtcacaaaagaacccagtctattgtaggggaaaaagtaaacactatatcagaaactctagagctacctaccatcagcaaacctgcacgatcatctacactgctagagccaaaattggcatgggcagacagcagcagagccaccaaaaccacagaaaaacaaacaaccaaaacaacagatcctgttgaagaagaggaactcaatgaaaagaagatatcaccttccagtgatgggaagactcccgcagagaaaaaatcaaaatctccaaccaatgtaaaaaagaaagtttccttcacatcaaatgaaccagggaaatataccaaactagaaaaagatgccctagatttgctctcagacaatgaggaagaagacgcagagtcctcaatcttaacctttgaagagagagacacatcatcactaagcattgaggctagactagaatcaatagaagagaagctaagcatgatattaggactgcttcgtacacttaacattgcaacagcaggaccaacggctgcaagagatggaatcagagatgcaatgattggtataagagaagaactaatagcagaaataataaaagaagcaaagggaaaagcagctgaaatgatggaagaggaaatgaatcaaaggtcaaaaataggtaatggcagtgtaaaactaaccgagaaggcaaaagaacttaataaaattgttgaagacgagagcacaagcggtgaatcagaagaagaagaagaaccaaaagaaactcaggataacaatcaaggagaagatatttaccagttaatcatgtagtttaataaaaataaacaatgggacaagtcaagatggagtcctatctagtggacacttatcaaggcattccctacacagctgctgttcaagttgatctggtagaaaaagacttactaccagcaagtttgacaatatggtttcctctattccaagccaacacaccaccagcggttttgctcgatcagctaaagaccttgacaataacaactctgtatgctgcatcacagaatggtccaatactcaaggtaaatgcatcagctcagggtgctgctatgtctgtacttcccaaaaaattcgaagtaaatgcaactgtggcacttgatgaatacagcaaacttgactttgacaagttaacggtttgcgatgttaaaacagtttatttgacaaccatgaaaccatatgggatggtgtcaaaatttgtgagttcagccaaatcagttggcaacaagacacatgatctaattgcactgtgtgacttcatggacctagagaaaaatatacctgtgacaataccagcattcataaagtcagtttcaatcaaagagagtgagtcagccactgttgaagctgcaataagcagtgaggccgaccaagcattaacacaagccaaaattgcaccctatgcaggactaatcatgatcatgaccatgaacaatccaaaaggtatattcaagaaactaggagctggaacacaagtgatagtagagctaggggcatatgttcaagccgagagcatcagcaggatctgcaagagctggagtcaccaaggaacaagatatgtactaaaatccagataaaaataactgtcctaatcaataattgcttatataatcttaaagatcaatgagcttattattatagttatataaaaaaatttagaactaggaaggtattaatagaaagcgggacaagtaaaaatgtcttggaaagtgatgattatcatttcgttactcataacacctcagcacggactaaaggaaagttatttagaagaatcatgtagtactataactgaaggatatctcagtgttttaagaacaggttggtacaccaatgtctttacattagaagttggtgatgttgaaaatcttacatgtactgatggacctagcttaatcaaaacagaacttgacctaaccaaaagtgctctaagagaactcaaaacagtttctgctgatcagttagcgagagaagaacaaattgaaaatcccagacaatcaaggtttgtcctaggtgcaatagctcttggtgttgccacagcagcagcagtcacagcaggcattgcgatagccaaaaccataaggcttgagagtgaagtgaatgcaatcaaaggtgctctcaaaacaaccaatgaggcagtatccacactaggaaatggagtgcgagtcctagccaccgcagtaagagagctgaaagaatttgtgagcaaaaacctgactagtgcaattaacaagaacaaatgtgacattgctgatctgaagatggctgtcagcttcagtcaattcaacagaagattcctaaatgttgtgcggcagttttcagacaatgcagggataacaccagcaatatcattggacctaatgactgatgctgagctggccagagctgtatcatacatgccaacatctgcaggacagataaaactaatgttagagaaccgtgcaatggtgaggagaaaaggatttggaatcttgataggggtctacggaagctccgtgatttacatggtccagctgccgatctttggtgtcatagatacaccttgttggataatcaaggcagctccctcttgttcagaaaaagatggaaactatgcttgcctcctaagagaggatcaagggtggtattgtaaaaatgcaggatccactgtttactacccaaataaaaaagactgcgaaacaagaggtgatcatgttttttgtgacacagctgcagggatcaatgttgctgagcaatcaagagaatgcaacatcaacatatctacaaccaactacccatgcaaagtcagcacaggaagacaccctatcagcatggttgcactatcacctctcggtgctttggtggcttgctacaaaggggttagctgttcaattggcagtaatcgggttggaataatcaaacaactacctaaaggctgctcatacataactaaccaggacgcagacactgtaacaattgacaacactgtgtatcaactaagcaaagttgagggtgaacagcatgtaataaaagggagaccagtttcaagcagtttcgatccaatcaagtttcctgaggatcagttcaatgttgcgcttgatcaagtctttgaaagcattgaaaacagtcaagcactagtggaccagtcaaacaaaattctgaacagtgcagaaaaaggaaacactggcttcattattgtaataattttgattgctgttcttgggttaaccatgatttcagtgagcatcatcatcataatcaaaaaaacaaggaaacccacaggggcacctccagagctgaatggtgttaccaacggcggttttataccgcatagttagttaattaaaaaatgggacaaatcatcatgtctcgtaaagctccatgcaaatatgaagtacggggcaagtgcaacaggggaagtgagtgcaaattcaaccacaattactggagttggcctgataggtatttattgttaagatcaaattatctcttgaatcagcttttaagaaacactgataaggctgatggtttgtcaataatatcaggagcaggtagagaagacaggactcaagactttgttcttggttctactaatgtggttcaagggtacattgatgacaatcaaggaataacaaaggctgcagcttgctatagtctacataacataataaaacagctacaagaaatagaagtaagacaggccagagataataagctttctgacagcaaacatgtggcacttcacaacttgatattatcctatatggagatgagcaaaactcctgcatccctgattaataacctaaagaaactaccaagagaaaaactgaaaaaattagcgaaattaataattgatttatcagcaggaactgataatgactcttcatatgccttgcaagacagtgaaagcactaatcaagtgcagtaagcatggtcccaaattcatcaccatagaggcagatgatatgatatggacacacaaagaattaaaagagacactgtctgatgggatagcaaaatcacacaccaatatttacagttgttatttagaaaatatagaaataatatatgttaaagcttacttaagttagtaaaaaataaatagaatgggataaatgacaatgaaaacattagatgtcataaaaagtgacggatcctcagaaacatgtaatcaactcaaaaaaataataaaaaaacactcaggtaaattgcttattgcatcaaaaccgacattggccttattgacgtccttcacagtaacaattactgtcaactatacaaaagtagaaaataatttgcaggcatgtcaattaaaaaatgaatcagacaaaaaggacacaaagctaaataccacatcaacaacaatcagacccattcctgatctaaatgcagtacagtacctgaaaaggctgattcagaaacacaccaactctgtcacaaaagacagagatacctgttggagaatacacacgaatcaatgcacaaatataaaaatatataagttcttatgttttgggtctatgaattcaacaaatacagactgtgaagaaccaacagttctatgcgacaaaaagtcaaaaaccatgacagaaaaacataggaaagcagagtgtcaccgtccacatacaaccgagtggtggtgccattatctttaagagaaaactcagttttcaacattaaaatcagaacaaatcatatctagatctattaatataatagtctagttatttaaaaactctaaatattgtctagacttcacaacaccctgcggtcatatgcaataatcaatggtcaaaccactgttgcaaacccacctataatacaatcactgagtaatacaaaacaagaaaatgggacaagtggccatggaagcaagagtggagaacattcgggcaatagacatgttcaaagcaaagatgaaaaaccgtataagaagtagcaagtgccatagaaatgctacactgatccttattggatcaacagcaccaagtatggcactcaacacccttttaatcattgatcatgcaacatcaaaaaacatgaccaaagtggaacactgtgtcaacatgccgccggtagaaccaagcaagaagaccccaatgacctctgcagcagacccaaacaccaaacccaatccacagcaggcaacacagctgaccacagaggattcaacatctctagcagcaaccctagaggaccatctacacacagggacaactccaacaccagatgcaacagtctcccagcaaaccacagacgagcacacaacactgctgagatcaaccaacagacagaccacccaaacaaccgcagagaaaaagccaaccagagcaacaaccaaaaaagaaaccacaactcgaaccacaagcacagctgcaacccaaacactcaacaccaccaaccaaactagcaatggaagagaggcaaccacaacatctgccagatccagaaacaatgccacaactcaaagcagcgatcaaacaacccaggcagcagacccaagctcccaatcacaacatacacagaaaagcacaacaacaacacacaacacagacacatcttctccaagtagttaacaaaaaaactataaaataaccatgaaaaccaaaaaactagaaaagttaatttgaactcagaaaagaacacaaacactatatgaattgtttgagcgtatatactaatgaaatagcatctgtttgtgcatcaataataccatcattatttaagaaataagaagaagctaaaattcaagggacaaataacaatggatccgttttgtgaatccactgtcaatgtctatcttcctgattcatatctcaaaggagtaatatctttcagtgaaaccaatgcaattggctcatgccttttgaaaagaccctatcttaaaaaagataacactgctaaagttgctgtagaaaaccctgttgttgaacatgtcagacttagaaatgcagtcatgaccaaaatgaagatatcagattataaagtggttgaaccaattaatatgcagcatgaaataatgaaaaatatacacagttgtgagctcacattattaaaacaattcttaacaagaagtaaaaacattagctccctaaaattaagtatgatatgtgattggttacagttaaaatccacctcagataacacatcaattcttaattttatagatgtggagtttatacccgtttgggtgagcaattggtttagtaactggtataatctcaataaattaatcttagagtttagaagagaggaagtaataagaactggttcaattttatgcagatcactaggcaagttagttttcattgtatcatcttatgggtgtgtagtaaaaagcaacaaaagtaaaagagtaagttttttcacatataaccaactgttaacatggaaagatgtgatgttaagtaggttcaatgcaaacttttgtatatgggtaagtaacaacctgaacaaaaatcaagaaggactaggatttagaagtaatctacaaggtatgttaactaataaattatatgaaactgttgattatatgttaagtctatgtagcaatgaagggttctcactagtgaaagagttcgaaggctttattatgagtgaaattcttaaaattactgagcatgctcaattcagtactaggtttaggaatactttattaaatgggttgactgaacaattatcaatgttgaaagctaaaaacagatctagagttcttggcactatattagaaaacaatgattaccccatgtatgaagtagtacttaaattattaggggacactttgaaaagtataaaattattaattaacaagaatttagaaaatgctgcagaattatattatatattcagaatttttggacaccctatggtagatgagagggaagcaatggatgctgttaaattaaataatgagattacaaaaattcttaaactggagagcttaacagaactaagaggagcatttatactaagaattataaaagggtttgtagataataataaaagatggcctaaaattaagaatttaaaagtgctcagtaaaagatgggttatgtatttcaaagctaaaagttaccctagccaacttgagctaagtgtacaagattttttagaacttgctgcagtacaattcgaacaggaattttctgtccctgaaaaaaccaatcttgagatggtattaaatgataaagcaatatctccaccaaaaaagttaatatggtcggtatatccaaaaaattatctacctgaaattataaaaaatcaatatttagaagaggtcttcaatgcaagtgacagtcaaagaacgaggagagtcttagaattttacttaaaagattgcaaatttgatcaaaaagacctcaaacgttatgtaactaaacaagagtatctaaatgacaaagaccacattgtctcattaactgggaaagaaagagaattaagtgtaggcaggatgtttgcaatgcaacctggcaaacaaagacaaatacagatactagccgagaaacttttagctgataatattgtaccctttttcccagaaactttaacaaagtatggtgacttggatctccaaagaattatggaaatgaaatcagaactttcttccattaaaactaggaagaatgatagttacaacaattatattgcaagagcctccatagtaacagacctaagtaaattcaatcaagcctttagatatgaaaccacagctatctgcgcagacgtagcagatgagttacatggcacgcaaagcttattttgttggttacatcttattgttcccatgaccacaatgatatgtgcatacagacatgcaccaccagaaacaaagggggagtatgatatagacaaaatagaagagcaaagtgggctatacagataccatatgggagggattgaagggtggtgtcagaagttatggacaatggaggcgatatccttgttagatgtagtatctgttaagactcgttgtcagatgacctctctattaaacggagacaatcaatcaatagatgtcagtaaaccagtaaaattgtctgaaggtatagatgaagtaaaagcagattatagcttagcaattaaaatgcttaaagagataagagatgcctataaaaacattggccataaactcaaagaaggtgaaacatatatatcaagagatcttcaatttataagtaaggtgattcaatctgagggggtcatgcatcctacccccataaaaaagatattaagggtaggtccctggataaatacaatactagatgacattaaaactagtgcagaatcaatagggagtctgtgtcaagaactagagttcagaggagaaagtatactagttagcttgatattaaggaatttctggctgtataacttatacatgcatgagtcaaaacagcatccgttagctggaaaacaactgtttaaacaattgaacaaaacactaacatctgtgcaaagattttttgagctgaagaaagaaaatgatgtggttgacctatggatgaatataccaatgcagtttggagggggagacccagtagttttttacagatctttttacagaaggactcctgatttcttgactgaagcaatcagccatgtggatttactgttaaaagtttcaaacaatattaaaaatgagactaagatacgattctttaaagccttattatctatagaaaagaatgaacgtgctacattaacaacactaatgagagacccccaggcggtaggatcggaaagacaagctaaggtaacaagtgatataaatagaacagcagttactagcatactgagtctatctccgaatcagctattttgtgatagtgctatacactatagcagaaatgaagaagaagtagggatcattgcagacaacataacacctgtttatcctcacggattgagagtgctctatgaatcactaccttttcataaggctgaaaaggttgtcaatatgatatcaggtacaaagtctataactaacctattgcagagaacatctgctatcaatggtgaagatattgatagagcagtgtctatgatgttagagaacttagggttgttatctaggatattgtcagtaataattaatagtatagaaataccaattaagtccaatggcagattgatatgctgtcaaatttctaagactttgagagaaaaatcatggaacaatatggaaatagtaggagtgacatctccaagtattgtaacatgtatggatgttgtgtatgcgactagttctcatttaaaaggaataattattgaaaaattcagtactgacaagaccacaagaggtcagaggggaccaaaaagcccttgggtaggatcaagcactcaagagaaaaaattagttcctgtttataacagacaaattctttcaaaacaacaaaaagagcaactggaagcaataggaaaaatgaggtgggtgtataaaggaactccagggctaagaagattgctcaataagatttgcataggaagtttaggtattagctataaatgtgtaaaacctctattaccaagatttatgagtgtaaacttcttacataggttatctgttagtagcagacccatggaattcccagcttctgttccagcttataggacaacaaattaccactttgacactagtccaatcaaccaagcattaagtgagaggttcgggaacgaagacattaatctagtgttccaaaatgcaatcagctgcggaattagtataatgagtgttgtagaacagttaactggtagaagcccaaaacaattagtcttaatcccccaattagaagagatagatattatgccccctcctgtatttcaaggaaaattcaattataaactagttgataaaataacctccgatcaacacatcttcagtcctgacaaaatagacatattaacactagggaagatgcttatgcctactataaaaggtcaaaaaactgatcagttcttaaataagagagaaaactatttccatggaaataatttaattgaatctttatctgcagcacttgcatgccattggtgtggaatattaacagaacagtgtgtagaaaacaatatctttaggaaagactggggtgatgggttcatatcagatcatgccttcatggatttcaagatatttctatgtgtatttaaaaccaaacttttatgtagttggggatcccaagggaaaaatgtaaaagatgaagatataatagatgaatccattgacaaattattaagaattgacaacactttttggagaatgttcagcaaagtcatgtttgaatcaaaggtcaaaaaaagaataatgttatatgatgtaaaattcctatcattagtaggttatataggatttaaaaactggtttatagagcagttaagagtagtagaattgcatgaagtaccctggattgtcaatgctgaaggggagctagttgaaattaaaccaatcaaaatttatttgcagttaatagaacaaagtctatctttaagaataactgttttgaattatacagacatggcacatgctcttacacgattaattaggaagaaattgatgtgtgataatgcactctttaatccaagttcatcaccaatgtttagtctaactcaagttattgatcctacaacacagctagactattttcctaaggtaatatttgaaaggttaaaaagttatgacaccagttcagactacaacaaagggaagttaacaagaaattacatgacattattaccatggcagcacgtaaacaggtataattttgtctttagttcaacaggatgtaaaatcagcttgaagacatgcatcgggaaattgataaaggacttaaaccctaaggttctttactttattggagaaggagcaggtaactggatggcaagaacagcatgtgagtatcctgacataaaatttgtatataggagtttaaaggatgatcttgatcaccattacccattagaatatcaaagggtaataggtgatttaaatagagtaatagatggtggtgaaggattatcaatggagaccacagatgcaactcaaaagactcattgggacttgatacacagaataagtaaagatgctttattgataacattgtgtgatgcagaattcaaaaacagagatgatttctttaaaatggtaattctttggagaaaacatgtattatcatgtagaatctgtacagcttatggaacagatctttacttatttgcaaagtatcatgcgacggactgcaatataaagttaccattttttgtaaggtctgtagctacttttattatgcaaggaagcaaattgtcaggatcagaatgttacatacttttaacattaggtcatcacaataatctgccatgtcacggagaaatacaaaattccaaaatgagaatagcagtgtgtaatgatttccatgcctcaaaaaaactagacaacaaatcaattgaagcaaactgcaaatctcttctatcaggattaagaataccaataaacaaaaaagagttaaatagacaaaagaaactgttaacactacaaagcaatcattcttccatagcaacagttggcggaagtaagattatagaatccaaatggttaaagaataaagcaagtacaataattgattggttagagcatatcttgaattctccaagaggtgaattaaactatgatttctttgaagcattagagaacacatatcccaatatgatcaagcttatagataacctgggaaatgcagagataaaaaaactaatcaaagttaccgggtatatgcttgtgagtgagaagtaataataataataataatcaaccataatctcacacaactgagaaaatgatcatctaacagtttaattgaccattagttaattaaaaattataaattagtaactaattgataaaaaataagaaattgaaattgaatgtatacggtttttttgccgt

SEQ ID NO: 8 - DNA, 14028 bp, Artificial Sequence
  Le gène de la GFP est inséré entre les positions 41 et 785
acgcgaaaaaaacgcgtataaattaaattccaaacaaaacgggacaaataaaaatggtgagcaagggcgaggagctgttcaccggggtggtgcccatcctggtcgagctggacggcgacgtaaacggccacaagttcagcgtgtccggcgagggcgagggcgatgccacctacggcaagctgaccctgaagttcatctgcaccaccggcaagctgcccgtgccctggcccaccctcgtgaccaccctgacctacggcgtgcagtgcttcagccgctaccccgaccacatgaagcagcacgacttcttcaagtccgccatgcccgaaggctacgtccaggagcgcaccatcttcttcaaggacgacggcaactacaagacccgcgccgaggtgaagttcgagggcgacaccctggtgaaccgcatcgagctgaagggcatcgacttcaaggaggacggcaacatcctggggcacaagctggagtacaactacaacagccacaacgtctatatcatggccgacaagcagaagaacggcatcaaggtgaacttcaagatccgccacaacatcgaggacggcagcgtgcagctcgccgaccactaccagcagaacacccccatcggcgacggccccgtgctgctgcccgacaaccactacctgagcacccagtccgccctgagcaaagaccccaacgagaagcgcgatcacatggtcctgctggagttcgtgaccgccgccgggatcactctcggcatggacgagctgtacaagtaagttaattaaaaaactgggacaaataaaaatgtctcttcaagggattcacctaagtgatctgtcatataaacatgctatattaaaagagtctcaatacacaataaaaagagatgtaggcaccacaactgcagtgacaccttcatcattgcagcaagagataacacttttgtgtggagagattctttacactaaacatactgattacaaatatgctgcagagatagggatacaatatatttgcacggctctaggatcagaaagagtacaacagattttaagaaattcaggcagtgaagttcaggtggttctaaccaagacatactctttagggaaaggtaaaaatagtaaaggggaagagttgcaaatgttagatatacatggagtggaaaagagttgggtagaagaaatagacaaagaggcaagaaaaacaatggtgactttgctaaaggaatcatcaggtaacatcccacaaaaccagaggccttcagcaccagacacaccaataattttattatgtgtaggtgctttaatattcactaaactagcatcaacaatagaagttggactagagactacagttagaagagctaacagagtgctaagtgatgcgctcaaaagataccctagggtagatataccgaagattgctagatctttctatgaactatttgagcagaaagtgtattacaggagtctattcattgagtatgggaaagctttaggctcatcttcaacaggaagcaaagcagaaagtttgtttgtaaatatatttatgcaagcttatggagccggtcaaacaatgctaaggtggggtgtcattgccagatcatctaacaacataatgctaggacatgtgtctgtgcaagctgaattgaagcaagttacagaggtttatgatttggtgagagaaatgggtcctgaatctgggcttttacatctaagacaaagtccaaaggcaggactgttatcgttggccaattgccccaattttgctagtgttgttcttggtaatgcttcaggtctaggtataatcggaatgtacagaggaagagtgccaaacacagagctattttctgcagcagaaagttatgccagaagcttaaaagaaagcaacaaaatcaacttctcctcattagggctcacagacgaagaaaaagaagctgcagaacacttcttaaacatgagtgatgacaatcaagatgattatgagtaattaaaaaactgggacaagtcaaaatgtcattccctgaaggaaaagatatcctgttcatgggtaatgaagcagcaaaaatagcagaagctttccagaaatcactaaaaagatcaggtcacaaaagaacccagtctattgtaggggaaaaagtaaacactatatcagaaactctagagctacctaccatcagcaaacctgcacgatcatctacactgctagagccaaaattggcatgggcagacagcagcagagccaccaaaaccacagaaaaacaaacaaccaaaacaacagatcctgttgaagaagaggaactcaatgaaaagaagatatcaccttccagtgatgggaagactcccgcagagaaaaaatcaaaatctccaaccaatgtaaaaaagaaagtttccttcacatcaaatgaaccagggaaatataccaaactagaaaaagatgccctagatttgctctcagacaatgaggaagaagacgcagagtcctcaatcttaacctttgaagagagagacacatcatcactaagcattgaggctagactagaatcaatagaagagaagctaagcatgatattaggactgcttcgtacacttaacattgcaacagcaggaccaacggctgcaagagatggaatcagagatgcaatgattggtataagagaagaactaatagcagaaataataaaagaagcaaagggaaaagcagctgaaatgatggaagaggaaatgaatcaaaggtcaaaaataggtaatggcagtgtaaaactaaccgagaaggcaaaagaacttaataaaattgttgaagacgagagcacaagcggtgaatcagaagaagaagaagaaccaaaagaaactcaggataacaatcaaggagaagatatttaccagttaatcatgtagtttaataaaaataaacaatgggacaagtcaagatggagtcctatctagtggacacttatcaaggcattccctacacagctgctgttcaagttgatctggtagaaaaagacttactaccagcaagtttgacaatatggtttcctctattccaagccaacacaccaccagcggttttgctcgatcagctaaagaccttgacaataacaactctgtatgctgcatcacagaatggtccaatactcaaggtaaatgcatcagctcagggtgctgctatgtctgtacttcccaaaaaattcgaagtaaatgcaactgtggcacttgatgaatacagcaaacttgactttgacaagttaacggtttgcgatgttaaaacagtttatttgacaaccatgaaaccatatgggatggtgtcaaaatttgtgagttcagccaaatcagttggcaacaagacacatgatctaattgcactgtgtgacttcatggacctagagaaaaatatacctgtgacaataccagcattcataaagtcagtttcaatcaaagagagtgagtcagccactgttgaagctgcaataagcagtgaggccgaccaagcattaacacaagccaaaattgcaccctatgcaggactaatcatgatcatgaccatgaacaatccaaaaggtatattcaagaaactaggagctggaacacaagtgatagtagagctaggggcatatgttcaagccgagagcatcagcaggatctgcaagagctggagtcaccaaggaacaagatatgtactaaaatccagataaaaataactgtcctaatcaataattgcttatataatcttaaagatcaatgagcttattattatagttatataaaaaaatttagaactaggaaggtattaatagaaagcgggacaagtaaaaatgtcttggaaagtgatgattatcatttcgttactcataacacctcagcacggactaaaggaaagttatttagaagaatcatgtagtactataactgaaggatatctcagtgttttaagaacaggttggtacaccaatgtctttacattagaagttggtgatgttgaaaatcttacatgtactgatggacctagcttaatcaaaacagaacttgacctaaccaaaagtgctctaagagaactcaaaacagtttctgctgatcagttagcgagagaagaacaaattgaaaatcccagacaatcaaggtttgtcctaggtgcaatagctcttggtgttgccacagcagcagcagtcacagcaggcattgcgatagccaaaaccataaggcttgagagtgaagtgaatgcaatcaaaggtgctctcaaaacaaccaatgaggcagtatccacactaggaaatggagtgcgagtcctagccaccgcagtaagagagctgaaagaatttgtgagcaaaaacctgactagtgcaattaacaagaacaaatgtgacattgctgatctgaagatggctgtcagcttcagtcaattcaacagaagattcctaaatgttgtgcggcagttttcagacaatgcagggataacaccagcaatatcattggacctaatgactgatgctgagctggccagagctgtatcatacatgccaacatctgcaggacagataaaactaatgttagagaaccgtgcaatggtgaggagaaaaggatttggaatcttgataggggtctacggaagctccgtgatttacatggtccagctgccgatctttggtgtcatagatacaccttgttggataatcaaggcagctccctcttgttcagaaaaagatggaaactatgcttgcctcctaagagaggatcaagggtggtattgtaaaaatgcaggatccactgtttactacccaaatgaaaaagactgcgaaacaagaggtgatcatgttttttgtgacacagctgcagggatcaatgttgctgagcaatcaagagaatgcaacatcaacatatctacaaccaactacccatgcaaagtcagcacaggaagacaccctatcagcatggttgcactatcacctctcggtgctttggtggcttgctacaaaggggttagctgttcaattggcagtaatcgggttggaataatcaaacaactacctaaaggctgctcatacataactaaccaggacgcagacactgtaacaattgacaacactgtgtatcaactaagcaaagttgagggtgaacagcatgtaataaaagggagaccagtttcaagcagtttcgatccaatcaagtttcctgaggatcagttcaatgttgcgcttgatcaagtctttgaaagcattgaaaacagtcaagcactagtggaccagtcaaacaaaattctgaacagtgcagaaaaaggaaacactggcttcattattgtaataattttgattgctgttcttgggttaaccatgatttcagtgagcatcatcatcataatcaaaaaaacaaggaaacccacaggggcacctccagagctgaatggtgttaccaacggcggttttataccgcatagttagttaattaaaaaatgggacaaatcatcatgtctcgtaaagctccatgcaaatatgaagtacggggcaagtgcaacaggggaagtgagtgcagattcaaccacaattactggagttggcctgataggtatttattgttaagatcaaattatctcttgaatcagcttttaagaaacactgataaggctgatggtttgtcaataatatcaggagcaggtagagaagacaggactcaagactttgttcttggttctactaatgtggttcaagggtacattgatgacaatcaaggaataacaaaggctgcagcttgctatagtctacataacataataaaacagctacaagaaatagaagtaagacaggccagagataataagctttctgacagcaaacatgtggcacttcacaacttgatattatcctatatggagatgagcaaaactcctgcatccctgattaataacctaaagaaactaccaagagaaaaactgaaaaaattagcgaaattaataattgatttatcagcaggaactgataatgactcttcatatgccttgcaagacagtgaaagcactaatcaagtgcagtaagcatggtcccaaattcattaccatagaggcagatgatatgatatggacacacaaagaattaaaagagacactgtctgatgggatagtaaaatcacacaccaatatttacagttgttatttagaaaatatagaaataatatatgttaaagcttacttaagttagtaaaaaataaatagaatgggataaatgacaatgaaaacattagatgtcataaaaagtgacggatcctcagaaacatgtaatcaactcaaaaaaataataaaaaaacactcaggtaaattgcttattgcattaaaactgatattggccttattgacgtttttcacagtaacaattactgttaactatataaaagtagaaaataatttgcaggcatgtcaattaaaaaatgaatcagacaaaaaggacacaaagctaaataccacatcaacaacaatcagacccattcctgatctaaatgcagtacagtacttgaaaaggctgattcagaaacacaccaactttgtcataaaagacagagatacctgttggagaatacacacgaatcaatgcacaaatataaaaatatataagttcttatgttttgggtctatgaattcaacaaatacagactgtgaagaactaacagttttatgcgacaaaaagtcaaaaaccatgacagaaaaacataggaaagcagagtgtcactgtctacatacaaccgagtggtggtgttattatctttaagagaaaactcagttttcaacattaaaatcagaacaaatcatatctagatctattaatataatagtttagttatttaaaaactctaaatattgtctagacttcacaacactttgcggtcatatgcaataatcaatggtcaaaccactgttgcaaactcacctataatataatcactgagtaatacaaaacaagaaaatgggacaagtggccatggaagtaagagtggagaacattcgggcaatagacatgttcaaagcaaagatgaaaaaccgtataagaagtagcaagtgctatagaaatgctacactgatccttattggatcaacagcactaagtatggcactcaatatttttttaatcattgattatgcaacatcaaaaaacatgaccaaagtggaacactgtgtcaatatgccgccggtagaaccaagcaagaagaccccaatgacctctgcagtagacccaaacaccaaacccaatccacagcaggcaacacagctgaccacagaggattcaacatctctagcagcaaccctagaggaccatctacacacagggacaactccaacaccagatgcaacagtctctcagcaaaccacagacgagcacacaacactgctgagatcaaccaacagacagaccacccaaacaaccgcagagaaaaagccaaccagagcaacaaccaaaaaagaaaccacaactcgaaccacaagcacagctgcaacccaaacactcaacaccaccaaccaaactagcaatggaagagaggcaaccacaacatctgccagatccagaaacaatgccacaactcaaagcagcgatcaaacaacccaggcagcagacccaagctcccaatcacaacatacacagaaaagcacaacaacaacacacaacacagacacatcttctccaagtagttaacaaaaaaactataaaataaccatgaaaaccaaaaaactagaaaagttaatttgaactcagaaaagaacacaaacactatatgaattgtttgagcgtatatactaatgaaatagcatctgtttgtgcatcaataataccatcattatttaagaaataagaagaagctaaaattcaagggacaaataacaatggatccgttttgtgaatccactgtcaatgtctatcttcctgattcatatctcaaaggagtaatatctttcagtgaaaccaatgcaattggctcatgccttttgaaaagaccctatcttaaaaaagataacactgctaaagttgctgtagaaaaccctgttgttgaacatgtcagacttagaaatgcagtcatgaccaaaatgaagatatcagattataaagtggttgaaccaattaatatgcagcatgaaataatgaaaaatatacacagttgtgagctcacattattaaaacaattcttaacaagaagtaaaaacattagctccctaaaattaagtatgatatgtgattggttacagttaaaatccacctcagataacacatcaattcttaattttatagatgtggagtttatacccgtttgggtgagcaattggtttagtaactggtataatctcaataaattaatcttagagtttagaagagaggaagtaataagaactggttcaattttatgcagatcactaggcaagttagttttcattgtatcatcttatgggtgtgtagtaaaaagcaacaaaagtaaaagagtaagttttttcacatataaccaactgttaacatggaaagatgtgatgttaagtaggttcaatgcaaacttttgtatatgggtaagtaacaacctgaacaaaaatcaagaaggactaggatttagaagtaatctacaaggtatgttaactaataaattatatgaaactgttgattatatgttaagtctatgtagcaatgaagggttctcactagtgaaagagttcgaaggctttattatgagtgaaattcttaaaattactgagcatgctcaattcagtactaggtttaggaatactttattaaatgggttgactgaacaattatcaatgttgaaagctaaaaacagatctagagttcttggcactatattagaaaacaatgattaccccatgtatgaagtagtacttaaattattaggggacactttgaaaagtataaaattattaattaacaagaatttagaaaatgctgcagaattatattatatattcagaatttttggacaccctatggtagatgagagggaagcaatggatgctgttaaattaaataatgagattacaaaaattcttaaactggagagcttaacagaactaagaggagcatttatactaagaattataaaagggtttgtagataataataaaagatggcctaaaattaagaatttaaaagtgctcagtaaaagatgggttatgtatttcaaagctaaaagttaccctagccaacttgagctaagtgtacaagattttttagaacttgctgcagtacaattcgaacaggaattttctgtccctgaaaaaaccaatcttgagatggtattaaatgataaagcaatatctccaccaaaaaagttaatatggtcggtatatccaaaaaattatctacctgaaattataaaaaatcaatatttagaagaggtcttcaatgcaagtgacagtcaaagaacgaggagagtcttagaattttacttaaaagattgcaaatttgatcaaaaagacctcaaacgttatgtaactaaacaagagtatctaaatgacaaagaccacattgtctcattaactgggaaagaaagagaattaagtgtaggcaggatgtttgcaatgcaacctggcaaacaaagacaaatacagatactagccgagaaacttttagctgataatattgtaccctttttcccagaaactttaacaaagtatggtgacttggatctccaaagaattatggaaatgaaatcagaactttcttccattaaaactaggaagaatgatagttacaacaattatattgcaagagcctccatagtaacagacctaagtaaattcaatcaagcctttagatatgaaaccacagctatctgcgcagacgtagcagatgagttacatggcacgcaaagcttattttgttggttacatcttattgttcccatgaccacaatgatatgtgcatacagacatgcaccaccagaaacaaagggggagtatgatatagacaaaatagaagagcaaagtgggctatacagataccatatgggagggattgaagggtggtgtcagaagttatggacaatggaggcgatatccttgttagatgtagtatctgttaagactcgttgtcagatgacctctctattaaacggagacaatcaatcaatagatgtcagtaaaccagtaaaattgtctgaaggtatagatgaagtaaaagcagattatagcttagcaattaaaatgcttaaagagataagagatgcctataaaaacattggccataaactcaaagaaggtgaaacatatatatcaagagatcttcaatttataagtaaggtgattcaatctgagggggtcatgcatcctacccccataaaaaagatattaagggtaggtccctggataaatacaatactagatgacattaaaactagtgcagaatcaatagggagtctgtgtcaagaactagagttcagaggagaaagtatactagttagcttgatattaaggaatttctggctgtataacttatacatgcatgagtcaaaacagcatccgttagctggaaaacaactgtttaaacaattgaacaaaacactaacatctgtgcaaagattttttgagctgaagaaagaaaatgatgtggttgacctatggatgaatataccaatgcagtttggagggggagacccagtagttttttacagatctttttacagaaggactcctgatttcttgactgaagcaatcagccatgtggatttactgttaaaagtttcaaacaatattaaaaatgagactaagatacgattctttaaagccttattatctatagaaaagaatgaacgtgctacattaacaacactaatgagagacccccaggcggtaggatcggaaagacaagctaaggtaacaagtgatataaatagaacagcagttactagcatactgagtctatctccgaatcagctattttgtgatagtgctatacactatagcagaaatgaagaagaagtagggatcattgcagacaacataacacctgtttatcctcacggattgagagtgctctatgaatcactaccttttcataaggctgaaaaggttgtcaatatgatatcaggtacaaagtctataactaacctattgcagagaacatctgctatcaatggtgaagatattgatagagcagtgtctatgatgttagagaacttagggttgttatctaggatattgtcagtaataattaatagtatagaaataccaattaagtccaatggcagattgatatgctgtcaaatttctaagactttgagagaaaaatcatggaacaatatggaaatagtaggagtgacatctccaagtattgtaacatgtatggatgttgtgtatgcgactagttctcatttaaaaggaataattattgaaaaattcagtactgacaagaccacaagaggtcagaggggaccaaaaagcccttgggtaggatcaagcactcaagagaaaaaattagttcctgtttataacagacaaattctttcaaaacaacaaaaagagcaactggaagcaataggaaaaatgaggtgggtgtataaaggaactccagggctaagaagattgctcaataagatttgcataggaagtttaggtattagctataaatgtgtaaaacctctattaccaagatttatgagtgtaaacttcttacataggttatctgttagtagcagacccatggaattcccagcttctgttccagcttataggacaacaaattaccactttgacactagtccaatcaaccaagcattaagtgagaggttcgggaacgaagacattaatctagtgttccaaaatgcaatcagctgcggaattagtataatgagtgttgtagaacagttaactggtagaagcccaaaacaattagtcttaatcccccaattagaagagatagatattatgccccctcctgtatttcaaggaaaattcaattataaactagttgataaaataacctccgatcaacacatcttcagtcctgacaaaatagacatattaacactagggaagatgcttatgcctactataaaaggtcaaaaaactgatcagttcttaaataagagagaaaactatttccatggaaataatttaattgaatctttatctgcagcacttgcatgccattggtgtggaatattaacagaacagtgtgtagaaaacaatatctttaggaaagactggggtgatgggttcatatcagatcatgccttcatggatttcaagatatttctatgtgtatttaaaaccaaacttttatgtagttggggatcccaagggaaaaatgtaaaagatgaagatataatagatgaatccattgacaaattattaagaattgacaacactttttggagaatgttcagcaaagtcatgtttgaatcaaaggtcaaaaaaagaataatgttatatgatgtaaaattcctatcattagtaggttatataggatttaaaaactggtttatagagcagttaagagtagtagaattgcatgaagtaccctggattgtcaatgctgaaggggagctagttgaaattaaaccaatcaaaatttatttgcagttaatagaacaaagtctatctttaagaataactgttttgaattatacagacatggcacatgctcttacacgattaattaggaagaaattgatgtgtgataatgcactctttaatccaagttcatcaccaatgtttagtctaactcaagttattgatcctacaacacagctagactattttcctaaggtaatatttgaaaggttaaaaagttatgacaccagttcagactacaacaaagggaagttaacaagaaattacatgacattattaccatggcagcacgtaaacaggtataattttgtctttagttcaacaggatgtaaaatcagcttgaagacatgcatcgggaaattgataaaggacttaaaccctaaggttctttactttattggagaaggagcaggtaactggatggcaagaacagcatgtgagtatcctgacataaaatttgtatataggagtttaaaggatgatcttgatcaccattacccattagaatatcaaagggtaataggtgatttaaatagagtaatagatggtggtgaaggattatcaatggagaccacagatgcaactcaaaagactcattgggacttgatacacagaataagtaaagatgctttattgataacattgtgtgatgcagaattcaaaaacagagatgatttctttaaaatggtaattctttggagaaaacatgtattatcatgtagaatctgtacagcttatggaacagatctttacttatttgcaaagtatcatgcgacggactgcaatataaagttaccattttttgtaaggtctgtagctacttttattatgcaaggaagcaaattgtcaggatcagaatgttacatacttttaacattaggtcatcacaataatctgccatgtcacggagaaatacaaaattccaaaatgagaatagcagtgtgtaatgatttccatgcctcaaaaaaactagacaacaaatcaattgaagcaaactgcaaatctcttctatcaggattaagaataccaataaacaaaaaagagttaaatagacaaaagaaactgttaacactacaaagcaatcattcttccatagcaacagttggcggaagtaagattatagaatccaaatggttaaagaataaagcaagtacaataattgattggttagagcatatcttgaattctccaaaaggtgaattaaactatgatttctttgaagcattagagaacacatatcccaatatgatcaagcttatagataacctgggaaatgcagagataaaaaaactaatcaaagttaccgggtatatgcttgtgagtgagaagtaataataataataataatcaaccataatctcacacaactgagaaaatgatcatctaacagtttaattgaccattagttaattaaaaattataaattagtaactaattgataaaaaataagaaattgaaattgaatgtatacggtttttttgccgt